European Patent Specification EP 3 206 711 B1, published May 31, 2023. Title: ANTIBODY MOLECULES TO PD-L1 AND USES THEREOF. Applicant: NOVARTIS AG DANA-FARBER CANCER INSTITUTE, INC. PRESIDENT AND FELLOWS OF HARVARD COLLEGE. The sequence listing filed with the application follows.

SEQUENCE LISTING (362 sequences)

SEQ ID NO: 1 - protein, 5 aa, Artificial Sequence
  source: /note="Description of Artificial Sequence: Synthetic peptide"
SYWMY

SEQ ID NO: 2 - protein, 17 aa, Artificial Sequence
  source: /note="Description of Artificial Sequence: Synthetic peptide"
RIDPNSGSTKYNEKFKN

SEQ ID NO: 3 - protein, 11 aa, Artificial Sequence
  source: /note="Description of Artificial Sequence: Synthetic peptide"
DYRKGLYAMDY

SEQ ID NO: 4 - protein, 7 aa, Artificial Sequence
  source: /note="Description of Artificial Sequence: Synthetic peptide"
GYTFTSY

SEQ ID NO: 5 - protein, 6 aa, Artificial Sequence
  source: /note="Description of Artificial Sequence: Synthetic peptide"
DPNSGS

SEQ ID NO: 6 - protein, 120 aa, Artificial Sequence
  source: /note="Description of Artificial Sequence: Synthetic polypeptide"
QVHLQQPGAELVKPGASVKLSCKASGYTFTSYWMYWVKQGPGRGLEWIGRIDPNSGSTKYNEKFKNKATLTVDKSSSTAYMQLSSLTSEDSAVYYCARDYRKGLYAMDYWGQGTSVTVSS

SEQ ID NO: 7 - DNA, 360 bp, Artificial Sequence
  source: /note="Description of Artificial Sequence: Synthetic polynucleotide"
caggtccacctgcagcagcctggggctgagcttgtgaagcctggggcttcagtgaagctgtcctgcaaggcttctggctacaccttcaccagttactggatgtactgggtgaaacaggggcctggacgaggccttgagtggattggaaggattgatcctaatagtgggagtactaagtacaatgagaagttcaagaacaaggccacactgactgtagacaaatcctccagcacagcctacatgcagctcagcagcctgacatctgaggactctgcggtctattattgtgcaagggactatagaaaggggctctatgctatggactactggggtcaaggaacctcagtcaccgtctcctca

SEQ ID NO: 8 - protein, 107 aa, Artificial Sequence
  source: /note="Description of Artificial Sequence: Synthetic polypeptide"
DIVMTQSHKFMSTSVGDRVSITCKASQDVGTAVAWYQQKPGQSPKLLIYWASTRHTGVPDRFTGSGSGTDFTLTISNVQSEDLADYFCQQYNSYPLTFGAGSKLELK

SEQ ID NO: 9 - protein, 11 aa, Artificial Sequence
  source: /note="Description of Artificial Sequence: Synthetic peptide"
KASQDVGTAVA

SEQ ID NO: 10 - protein, 7 aa, Artificial Sequence
  source: /note="Description of Artificial Sequence: Synthetic peptide"
WASTRHT

SEQ ID NO: 11 - protein, 9 aa, Artificial Sequence
  source: /note="Description of Artificial Sequence: Synthetic peptide"
QQYNSYPLT

SEQ ID NO: 12 - protein, 7 aa, Artificial Sequence
  source: /note="Description of Artificial Sequence: Synthetic peptide"
SQDVGTA

SEQ ID NO: 13 - protein, 3 aa, Artificial Sequence
  source: /note="Description of Artificial Sequence: Synthetic peptide"
WAS

SEQ ID NO: 14 - protein, 6 aa, Artificial Sequence
  source: /note="Description of Artificial Sequence: Synthetic peptide"
YNSYPL

SEQ ID NO: 15 - DNA, 321 bp, Artificial Sequence
  source: /note="Description of Artificial Sequence: Synthetic polynucleotide"
gacattgtgatgacccagtctcacaaattcatgtccacatcagtaggagacagggtcagcatcacctgcaaggccagtcaggatgtgggtactgctgtagcctggtatcaacagaaaccagggcaatctcctaaactactgatttactgggcatccacccggcacactggagtccctgatcgcttcacaggcagtggatctgggacagatttcactctcaccattagcaatgtgcagtctgaagacttggcagattatttctgtcagcagtataacagctatcctctcacgttcggtgctgggtccaagctggagctgaaa

SEQ ID NO: 16 - protein, 120 aa, Artificial Sequence
  source: /note="Description of Artificial Sequence: Synthetic polypeptide"
EVQLQQSGAELVKPGASVKLSCKASGYTFTSYWMYWVKQGPGRGLEWIGRIDPNSGSTKYNEKFKNKATLTVDKSSSTAYMQLSSLTSEDSAVYYCARDYRKGLYAMDYWGQGTTVTVSS

SEQ ID NO: 17 - protein, 107 aa, Artificial Sequence
  source: /note="Description of Artificial Sequence: Synthetic polypeptide"
DIMMTQSHKFMSTSVGDRVSITCKASQDVGTAVAWYQQKPGQSPKLLIYWASTRHTGVPDRFTGSGSGTDFTLTISNVQSEDLADYFCQQYNSYPLTFGQGTKVEIK

SEQ ID NO: 18 - protein, 120 aa, Artificial Sequence
  source: /note="Description of Artificial Sequence: Synthetic polypeptide"
QVQLVQSGAEVKKPGASVKVSCKASGYTFTSYWMYWVRQATGQGLEWMGRIDPNSGSTKYNEKFKNRFTISRDDSKNTAYLQMNSLKTEDTAVYYCARDYRKGLYAMDYWGQGTTVTVSS

SEQ ID NO: 19 - DNA, 360 bp, Artificial Sequence
  source: /note="Description of Artificial Sequence: Synthetic polynucleotide"
caggttcagctggtgcagtctggagctgaggtgaagaagcctggggcctcagtgaaggtctcctgcaaggcttctggctacaccttcaccagttactggatgtactgggtgcgacaggccactggacaagggcttgagtggatgggtaggattgatcctaatagtgggagtactaagtacaatgagaagttcaagaacagattcaccatctccagagatgattcaaagaacacggcgtatctgcaaatgaacagcctgaaaaccgaggacacggccgtgtattactgtgcaagggactatagaaaggggctctatgctatggactactggggccagggcaccaccgtgaccgtgtcctcc

SEQ ID NO: 20 - protein, 447 aa, Artificial Sequence
  source: /note="Description of Artificial Sequence: Synthetic polypeptide"
QVQLVQSGAEVKKPGASVKVSCKASGYTFTSYWMYWVRQATGQGLEWMGRIDPNSGSTKYNEKFKNRFTISRDDSKNTAYLQMNSLKTEDTAVYYCARDYRKGLYAMDYWGQGTTVTVSSASTKGPSVFPLAPCSRSTSESTAALGCLVKDYFPEPVTVSWNSGALTSGVHTFPAVLQSSGLYSLSSVVTVPSSSLGTKTYTCNVDHKPSNTKVDKRVESKYGPPCPPCPAPEFLGGPSVFLFPPKPKDTLMISRTPEVTCVVVDVSQEDPEVQFNWYVDGVEVHNAKTKPREEQFNSTYRVVSVLTVLHQDWLNGKEYKCKVSNKGLPSSIEKTISKAKGQPREPQVYTLPPSQEEMTKNQVSLTCLVKGFYPSDIAVEWESNGQPENNYKTTPPVLDSDGSFFLYSRLTVDKSRWQEGNVFSCSVMHEALHNHYTQKSLSLSLGK

SEQ ID NO: 21 - DNA, 1341 bp, Artificial Sequence
  source: /note="Description of Artificial Sequence: Synthetic polynucleotide"
caggttcagctggtgcagtctggagctgaggtgaagaagcctggggcctcagtgaaggtctcctgcaaggcttctggctacaccttcaccagttactggatgtactgggtgcgacaggccactggacaagggcttgagtggatgggtaggattgatcctaatagtgggagtactaagtacaatgagaagttcaagaacagattcaccatctccagagatgattcaaagaacacggcgtatctgcaaatgaacagcctgaaaaccgaggacacggccgtgtattactgtgcaagggactatagaaaggggctctatgctatggactactggggccagggcaccaccgtgaccgtgtcctccgcttccaccaagggcccatccgtcttccccctggcgccctgctccaggagcacctccgagagcacagccgccctgggctgcctggtcaaggactacttccccgaaccggtgacggtgtcgtggaactcaggcgccctgaccagcggcgtgcacaccttcccggctgtcctacagtcctcaggactctactccctcagcagcgtggtgaccgtgccctccagcagcttgggcacgaagacctacacctgcaacgtagatcacaagcccagcaacaccaaggtggacaagagagttgagtccaaatatggtcccccatgcccaccgtgcccagcacctgagttcctggggggaccatcagtcttcctgttccccccaaaacccaaggacactctcatgatctcccggacccctgaggtcacgtgcgtggtggtggacgtgagccaggaagaccccgaggtccagttcaactggtacgtggatggcgtggaggtgcataatgccaagacaaagccgcgggaggagcagttcaacagcacgtaccgtgtggtcagcgtcctcaccgtcctgcaccaggactggctgaacggcaaggagtacaagtgcaaggtgtccaacaaaggcctcccgtcctccatcgagaaaaccatctccaaagccaaagggcagccccgagagccacaggtgtacaccctgcccccatcccaggaggagatgaccaagaaccaggtcagcctgacctgcctggtcaaaggcttctaccccagcgacatcgccgtggagtgggagagcaatgggcagccggagaacaactacaagaccacgcctcccgtgctggactccgacggctccttcttcctctacagcaggctaaccgtggacaagagcaggtggcaggaggggaatgtcttctcatgctccgtgatgcatgaggctctgcacaaccactacacacagaagagcctctccctgtctctgggtaaa

SEQ ID NO: 22 - protein, 107 aa, Artificial Sequence
  source: /note="Description of Artificial Sequence: Synthetic polypeptide"
DIVMTQTPLSLPVTPGEPASISCKASQDVGTAVAWYLQKPGQSPQLLIYWASTRHTGIPARFSGSGSGTEFTLTISSLQSEDFAVYYCQQYNSYPLTFGQGTKVEIK

SEQ ID NO: 23 - DNA, 321 bp, Artificial Sequence
  source: /note="Description of Artificial Sequence: Synthetic polynucleotide"
gatattgtgatgacccagactccactctccctgcccgtcacccctggagagccggcctccatctcctgcaaggccagtcaggatgtgggtactgctgtagcctggtacctgcagaagccagggcagtctccacagctcctgatctattgggcatccacccggcacactgggatcccagccaggttcagtggcagtgggtctgggacagagttcactctcaccatcagcagcctgcagtctgaagattttgcagtttattactgtcagcagtataacagctatcctctcacgttcggccaagggaccaaggtggaaatcaaa

SEQ ID NO: 24 - protein, 214 aa, Artificial Sequence
  source: /note="Description of Artificial Sequence: Synthetic polypeptide"
DIVMTQTPLSLPVTPGEPASISCKASQDVGTAVAWYLQKPGQSPQLLIYWASTRHTGIPARFSGSGSGTEFTLTISSLQSEDFAVYYCQQYNSYPLTFGQGTKVEIKRTVAAPSVFIFPPSDEQLKSGTASVVCLLNNFYPREAKVQWKVDNALQSGNSQESVTEQDSKDSTYSLSSTLTLSKADYEKHKVYACEVTHQGLSSPVTKSFNRGEC

SEQ ID NO: 25 - DNA, 642 bp, Artificial Sequence
  source: /note="Description of Artificial Sequence: Synthetic polynucleotide"
gatattgtgatgacccagactccactctccctgcccgtcacccctggagagccggcctccatctcctgcaaggccagtcaggatgtgggtactgctgtagcctggtacctgcagaagccagggcagtctccacagctcctgatctattgggcatccacccggcacactgggatcccagccaggttcagtggcagtgggtctgggacagagttcactctcaccatcagcagcctgcagtctgaagattttgcagtttattactgtcagcagtataacagctatcctctcacgttcggccaagggaccaaggtggaaatcaaacgtacggtggctgcaccatctgtcttcatcttcccgccatctgatgagcagttgaaatctggaactgcctctgttgtgtgcctgctgaataacttctatcccagagaggccaaagtacagtggaaggtggataacgccctccaatcgggtaactcccaggagagtgtcacagagcaggacagcaaggacagcacctacagcctcagcagcaccctgacgctgagcaaagcagactacgagaaacacaaagtctacgcctgcgaagtcacccatcagggcctgagctcgcccgtcacaaagagcttcaacaggggagagtgt

SEQ ID NO: 26 - protein, 107 aa, Artificial Sequence
  source: /note="Description of Artificial Sequence: Synthetic polypeptide"
DIQMTQSPSSLSASVGDRVTITCKASQDVGTAVAWYLQKPGQSPQLLIYWASTRHTGVPSRFSGSGSGTDFTLTISSLQPEDFATYYCQQYNSYPLTFGQGTKVEIK

SEQ ID NO: 27 - DNA, 321 bp, Artificial Sequence
  source: /note="Description of Artificial Sequence: Synthetic polynucleotide"
gacatccagatgacccagtctccatcctccctgtctgcatctgtaggagacagagtcaccatcacttgcaaggccagtcaggatgtgggtactgctgtagcctggtacctgcagaagccagggcagtctccacagctcctgatctattgggcatccacccggcacactggggtcccatcaaggttcagcggcagtggatctgggacagatttcactctcaccatcagcagcctgcagcctgaagattttgcaacttattactgtcagcagtataacagctatcctctcacgttcggccaagggaccaaggtggaaatcaaa

SEQ ID NO: 28 - protein, 214 aa, Artificial Sequence
  source: /note="Description of Artificial Sequence: Synthetic polypeptide"
DIQMTQSPSSLSASVGDRVTITCKASQDVGTAVAWYLQKPGQSPQLLIYWASTRHTGVPSRFSGSGSGTDFTLTISSLQPEDFATYYCQQYNSYPLTFGQGTKVEIKRTVAAPSVFIFPPSDEQLKSGTASVVCLLNNFYPREAKVQWKVDNALQSGNSQESVTEQDSKDSTYSLSSTLTLSKADYEKHKVYACEVTHQGLSSPVTKSFNRGEC

SEQ ID NO: 29 - DNA, 642 bp, Artificial Sequence
  source: /note="Description of Artificial Sequence: Synthetic polynucleotide"
gacatccagatgacccagtctccatcctccctgtctgcatctgtaggagacagagtcaccatcacttgcaaggccagtcaggatgtgggtactgctgtagcctggtacctgcagaagccagggcagtctccacagctcctgatctattgggcatccacccggcacactggggtcccatcaaggttcagcggcagtggatctgggacagatttcactctcaccatcagcagcctgcagcctgaagattttgcaacttattactgtcagcagtataacagctatcctctcacgttcggccaagggaccaaggtggaaatcaaacgtacggtggctgcaccatctgtcttcatcttcccgccatctgatgagcagttgaaatctggaactgcctctgttgtgtgcctgctgaataacttctatcccagagaggccaaagtacagtggaaggtggataacgccctccaatcgggtaactcccaggagagtgtcacagagcaggacagcaaggacagcacctacagcctcagcagcaccctgacgctgagcaaagcagactacgagaaacacaaagtctacgcctgcgaagtcacccatcagggcctgagctcgcccgtcacaaagagcttcaacaggggagagtgt

SEQ ID NO: 30 - protein, 120 aa, Artificial Sequence
  source: /note="Description of Artificial Sequence: Synthetic polypeptide"
EVQLVQSGAEVKKPGATVKISCKVSGYTFTSYWMYWVRQATGQGLEWMGRIDPNSGSTKYNEKFKNRVTITADKSTSTAYMELSSLRSEDTAVYYCARDYRKGLYAMDYWGQGTTVTVSS

SEQ ID NO: 31 - DNA, 360 bp, Artificial Sequence
  source: /note="Description of Artificial Sequence: Synthetic polynucleotide"
gaggtccagctggtacagtctggggctgaggtgaagaagcctggggctacagtgaaaatctcctgcaaggtttctggctacaccttcaccagttactggatgtactgggtgcgacaggccactggacaagggcttgagtggatgggtaggattgatcctaatagtgggagtactaagtacaatgagaagttcaagaacagagtcacgattaccgcggacaaatccacgagcacagcctacatggagctgagcagcctgagatctgaggacacggccgtgtattactgtgcaagggactatagaaaggggctctatgctatggactactggggccagggcaccaccgtgaccgtgtcctcc

SEQ ID NO: 32 - protein, 447 aa, Artificial Sequence
  source: /note="Description of Artificial Sequence: Synthetic polypeptide"
EVQLVQSGAEVKKPGATVKISCKVSGYTFTSYWMYWVRQATGQGLEWMGRIDPNSGSTKYNEKFKNRVTITADKSTSTAYMELSSLRSEDTAVYYCARDYRKGLYAMDYWGQGTTVTVSSASTKGPSVFPLAPCSRSTSESTAALGCLVKDYFPEPVTVSWNSGALTSGVHTFPAVLQSSGLYSLSSVVTVPSSSLGTKTYTCNVDHKPSNTKVDKRVESKYGPPCPPCPAPEFLGGPSVFLFPPKPKDTLMISRTPEVTCVVVDVSQEDPEVQFNWYVDGVEVHNAKTKPREEQFNSTYRVVSVLTVLHQDWLNGKEYKCKVSNKGLPSSIEKTISKAKGQPREPQVYTLPPSQEEMTKNQVSLTCLVKGFYPSDIAVEWESNGQPENNYKTTPPVLDSDGSFFLYSRLTVDKSRWQEGNVFSCSVMHEALHNHYTQKSLSLSLGK

SEQ ID NO: 33 - DNA, 1341 bp, Artificial Sequence
  source: /note="Description of Artificial Sequence: Synthetic polynucleotide"
gaggtccagctggtacagtctggggctgaggtgaagaagcctggggctacagtgaaaatctcctgcaaggtttctggctacaccttcaccagttactggatgtactgggtgcgacaggccactggacaagggcttgagtggatgggtaggattgatcctaatagtgggagtactaagtacaatgagaagttcaagaacagagtcacgattaccgcggacaaatccacgagcacagcctacatggagctgagcagcctgagatctgaggacacggccgtgtattactgtgcaagggactatagaaaggggctctatgctatggactactggggccagggcaccaccgtgaccgtgtcctccgcttccaccaagggcccatccgtcttccccctggcgccctgctccaggagcacctccgagagcacagccgccctgggctgcctggtcaaggactacttccccgaaccggtgacggtgtcgtggaactcaggcgccctgaccagcggcgtgcacaccttcccggctgtcctacagtcctcaggactctactccctcagcagcgtggtgaccgtgccctccagcagcttgggcacgaagacctacacctgcaacgtagatcacaagcccagcaacaccaaggtggacaagagagttgagtccaaatatggtcccccatgcccaccgtgcccagcacctgagttcctggggggaccatcagtcttcctgttccccccaaaacccaaggacactctcatgatctcccggacccctgaggtcacgtgcgtggtggtggacgtgagccaggaagaccccgaggtccagttcaactggtacgtggatggcgtggaggtgcataatgccaagacaaagccgcgggaggagcagttcaacagcacgtaccgtgtggtcagcgtcctcaccgtcctgcaccaggactggctgaacggcaaggagtacaagtgcaaggtgtccaacaaaggcctcccgtcctccatcgagaaaaccatctccaaagccaaagggcagccccgagagccacaggtgtacaccctgcccccatcccaggaggagatgaccaagaaccaggtcagcctgacctgcctggtcaaaggcttctaccccagcgacatcgccgtggagtgggagagcaatgggcagccggagaacaactacaagaccacgcctcccgtgctggactccgacggctccttcttcctctacagcaggctaaccgtggacaagagcaggtggcaggaggggaatgtcttctcatgctccgtgatgcatgaggctctgcacaaccactacacacagaagagcctctccctgtctctgggtaaa

SEQ ID NO: 34 - protein, 107 aa, Artificial Sequence
  source: /note="Description of Artificial Sequence: Synthetic polypeptide"
EIVLTQSPDFQSVTPKEKVTITCKASQDVGTAVAWYLQKPGQSPQLLIYWASTRHTGVPDRFSGSGSGTDFTLKISRVEAEDVGVYYCQQYNSYPLTFGQGTKVEIK

SEQ ID NO: 35 - DNA, 321 bp, Artificial Sequence
  source: /note="Description of Artificial Sequence: Synthetic polynucleotide"
gaaattgtgctgactcagtctccagactttcagtctgtgactccaaaggagaaagtcaccatcacctgcaaggccagtcaggatgtgggtactgctgtagcctggtacctgcagaagccagggcagtctccacagctcctgatctattgggcatccacccggcacactggggtcccagacaggttcagtggcagtgggtcaggcactgatttcacactgaaaatcagcagggtggaggctgaggatgttggagtttattactgtcagcagtataacagctatcctctcacgttcggccaagggaccaaggtggaaatcaaa

SEQ ID NO: 36 - protein, 214 aa, Artificial Sequence
  source: /note="Description of Artificial Sequence: Synthetic polypeptide"
EIVLTQSPDFQSVTPKEKVTITCKASQDVGTAVAWYLQKPGQSPQLLIYWASTRHTGVPDRFSGSGSGTDFTLKISRVEAEDVGVYYCQQYNSYPLTFGQGTKVEIKRTVAAPSVFIFPPSDEQLKSGTASVVCLLNNFYPREAKVQWKVDNALQSGNSQESVTEQDSKDSTYSLSSTLTLSKADYEKHKVYACEVTHQGLSSPVTKSFNRGEC

SEQ ID NO: 37 - DNA, 642 bp, Artificial Sequence
  source: /note="Description of Artificial Sequence: Synthetic polynucleotide"
gaaattgtgctgactcagtctccagactttcagtctgtgactccaaaggagaaagtcaccatcacctgcaaggccagtcaggatgtgggtactgctgtagcctggtacctgcagaagccagggcagtctccacagctcctgatctattgggcatccacccggcacactggggtcccagacaggttcagtggcagtgggtcaggcactgatttcacactgaaaatcagcagggtggaggctgaggatgttggagtttattactgtcagcagtataacagctatcctctcacgttcggccaagggaccaaggtggaaatcaaacgtacggtggctgcaccatctgtcttcatcttcccgccatctgatgagcagttgaaatctggaactgcctctgttgtgtgcctgctgaataacttctatcccagagaggccaaagtacagtggaaggtggataacgccctccaatcgggtaactcccaggagagtgtcacagagcaggacagcaaggacagcacctacagcctcagcagcaccctgacgctgagcaaagcagactacgagaaacacaaagtctacgcctgcgaagtcacccatcagggcctgagctcgcccgtcacaaagagcttcaacaggggagagtgt

SEQ ID NO: 38 - protein, 120 aa, Artificial Sequence
  source: /note="Description of Artificial Sequence: Synthetic polypeptide"
EVQLVQSGAEVKKPGESLRISCKGSGYTFTSYWMYWVRQAPGQGLEWMGRIDPNSGSTKYNEKFKNRVTISVDTSKNQFSLKLSSVTAADTAVYYCARDYRKGLYAMDYWGQGTTVTVSS

SEQ ID NO: 39 - DNA, 360 bp, Artificial Sequence
  source: /note="Description of Artificial Sequence: Synthetic polynucleotide"
gaagtgcagctggtgcagtctggagcagaggtgaaaaagcccggggagtctctgaggatctcctgtaagggttctggctacaccttcaccagttactggatgtactgggtgcgacaggcccctggacaagggcttgagtggatgggtaggattgatcctaatagtgggagtactaagtacaatgagaagttcaagaacagagtcaccatatcagtagacacgtccaagaaccagttctccctgaagctgagctctgtgaccgccgcggacacggctgtgtattactgtgcaagggactatagaaaggggctctatgctatggactactggggccagggcaccaccgtgaccgtgtcctcc

SEQ ID NO: 40 - protein, 447 aa, Artificial Sequence
  source: /note="Description of Artificial Sequence: Synthetic polypeptide"
EVQLVQSGAEVKKPGESLRISCKGSGYTFTSYWMYWVRQAPGQGLEWMGRIDPNSGSTKYNEKFKNRVTISVDTSKNQFSLKLSSVTAADTAVYYCARDYRKGLYAMDYWGQGTTVTVSSASTKGPSVFPLAPCSRSTSESTAALGCLVKDYFPEPVTVSWNSGALTSGVHTFPAVLQSSGLYSLSSVVTVPSSSLGTKTYTCNVDHKPSNTKVDKRVESKYGPPCPPCPAPEFLGGPSVFLFPPKPKDTLMISRTPEVTCVVVDVSQEDPEVQFNWYVDGVEVHNAKTKPREEQFNSTYRVVSVLTVLHQDWLNGKEYKCKVSNKGLPSSIEKTISKAKGQPREPQVYTLPPSQEEMTKNQVSLTCLVKGFYPSDIAVEWESNGQPENNYKTTPPVLDSDGSFFLYSRLTVDKSRWQEGNVFSCSVMHEALHNHYTQKSLSLSLGK

SEQ ID NO: 41 - DNA, 1341 bp, Artificial Sequence
  source: /note="Description of Artificial Sequence: Synthetic polynucleotide"
gaagtgcagctggtgcagtctggagcagaggtgaaaaagcccggggagtctctgaggatctcctgtaagggttctggctacaccttcaccagttactggatgtactgggtgcgacaggcccctggacaagggcttgagtggatgggtaggattgatcctaatagtgggagtactaagtacaatgagaagttcaagaacagagtcaccatatcagtagacacgtccaagaaccagttctccctgaagctgagctctgtgaccgccgcggacacggctgtgtattactgtgcaagggactatagaaaggggctctatgctatggactactggggccagggcaccaccgtgaccgtgtcctccgcttccaccaagggcccatccgtcttccccctggcgccctgctccaggagcacctccgagagcacagccgccctgggctgcctggtcaaggactacttccccgaaccggtgacggtgtcgtggaactcaggcgccctgaccagcggcgtgcacaccttcccggctgtcctacagtcctcaggactctactccctcagcagcgtggtgaccgtgccctccagcagcttgggcacgaagacctacacctgcaacgtagatcacaagcccagcaacaccaaggtggacaagagagttgagtccaaatatggtcccccatgcccaccgtgcccagcacctgagttcctggggggaccatcagtcttcctgttccccccaaaacccaaggacactctcatgatctcccggacccctgaggtcacgtgcgtggtggtggacgtgagccaggaagaccccgaggtccagttcaactggtacgtggatggcgtggaggtgcataatgccaagacaaagccgcgggaggagcagttcaacagcacgtaccgtgtggtcagcgtcctcaccgtcctgcaccaggactggctgaacggcaaggagtacaagtgcaaggtgtccaacaaaggcctcccgtcctccatcgagaaaaccatctccaaagccaaagggcagccccgagagccacaggtgtacaccctgcccccatcccaggaggagatgaccaagaaccaggtcagcctgacctgcctggtcaaaggcttctaccccagcgacatcgccgtggagtgggagagcaatgggcagccggagaacaactacaagaccacgcctcccgtgctggactccgacggctccttcttcctctacagcaggctaaccgtggacaagagcaggtggcaggaggggaatgtcttctcatgctccgtgatgcatgaggctctgcacaaccactacacacagaagagcctctccctgtctctgggtaaa

SEQ ID NO: 42 - protein, 107 aa, Artificial Sequence
  source: /note="Description of Artificial Sequence: Synthetic polypeptide"
EIVLTQSPDFQSVTPKEKVTITCKASQDVGTAVAWYLQKPGQSPQLLIYWASTRHTGVPSRFSGSGSGTDFTFTISSLQPEDIATYYCQQYNSYPLTFGQGTKVEIK

SEQ ID NO: 43 - DNA, 321 bp, Artificial Sequence
  source: /note="Description of Artificial Sequence: Synthetic polynucleotide"
gaaattgtgctgactcagtctccagactttcagtctgtgactccaaaggagaaagtcaccatcacctgcaaggccagtcaggatgtgggtactgctgtagcctggtacctgcagaagccagggcagtctccacagctcctgatctattgggcatccacccggcacactggggtcccatcaaggttcagtggaagtggatctgggacagattttactttcaccatcagcagcctgcagcctgaagatattgcaacatattactgtcagcagtataacagctatcctctcacgttcggccaagggaccaaggtggaaatcaaa

SEQ ID NO: 44 - protein, 214 aa, Artificial Sequence
  source: /note="Description of Artificial Sequence: Synthetic polypeptide"
EIVLTQSPDFQSVTPKEKVTITCKASQDVGTAVAWYLQKPGQSPQLLIYWASTRHTGVPSRFSGSGSGTDFTFTISSLQPEDIATYYCQQYNSYPLTFGQGTKVEIKRTVAAPSVFIFPPSDEQLKSGTASVVCLLNNFYPREAKVQWKVDNALQSGNSQESVTEQDSKDSTYSLSSTLTLSKADYEKHKVYACEVTHQGLSSPVTKSFNRGEC

SEQ ID NO: 45 - DNA, 642 bp, Artificial Sequence
  source: /note="Description of Artificial Sequence: Synthetic polynucleotide"
gaaattgtgctgactcagtctccagactttcagtctgtgactccaaaggagaaagtcaccatcacctgcaaggccagtcaggatgtgggtactgctgtagcctggtacctgcagaagccagggcagtctccacagctcctgatctattgggcatccacccggcacactggggtcccatcaaggttcagtggaagtggatctgggacagattttactttcaccatcagcagcctgcagcctgaagatattgcaacatattactgtcagcagtataacagctatcctctcacgttcggccaagggaccaaggtggaaatcaaacgtacggtggctgcaccatctgtcttcatcttcccgccatctgatgagcagttgaaatctggaactgcctctgttgtgtgcctgctgaataacttctatcccagagaggccaaagtacagtggaaggtggataacgccctccaatcgggtaactcccaggagagtgtcacagagcaggacagcaaggacagcacctacagcctcagcagcaccctgacgctgagcaaagcagactacgagaaacacaaagtctacgcctgcgaagtcacccatcagggcctgagctcgcccgtcacaaagagcttcaacaggggagagtgt

SEQ ID NO: 46 - protein, 120 aa, Artificial Sequence
  source: /note="Description of Artificial Sequence: Synthetic polypeptide"
EVQLVQSGAEVKKPGATVKISCKVSGYTFTSYWMYWIRQSPSRGLEWLGRIDPNSGSTKYNEKFKNRLTISKDTSKNQVVLTMTNMDPVDTATYYCARDYRKGLYAMDYWGQGTTVTVSS

SEQ ID NO: 47 - DNA, 360 bp, Artificial Sequence
  source: /note="Description of Artificial Sequence: Synthetic polynucleotide"
gaggtccagctggtacagtctggggctgaggtgaagaagcctggggctacagtgaaaatctcctgcaaggtttctggctacaccttcaccagttactggatgtactggatcaggcagtccccatcgagaggccttgagtggctgggtaggattgatcctaatagtgggagtactaagtacaatgagaagttcaagaacagactcaccatctccaaggacacctccaaaaaccaggtggtccttacaatgaccaacatggaccctgtggacacagccacgtattactgtgcaagggactatagaaaggggctctatgctatggactactggggccagggcaccaccgtgaccgtgtcctcc

SEQ ID NO: 48 - protein, 447 aa, Artificial Sequence
  source: /note="Description of Artificial Sequence: Synthetic polypeptide"
EVQLVQSGAEVKKPGATVKISCKVSGYTFTSYWMYWIRQSPSRGLEWLGRIDPNSGSTKYNEKFKNRLTISKDTSKNQVVLTMTNMDPVDTATYYCARDYRKGLYAMDYWGQGTTVTVSSASTKGPSVFPLAPCSRSTSESTAALGCLVKDYFPEPVTVSWNSGALTSGVHTFPAVLQSSGLYSLSSVVTVPSSSLGTKTYTCNVDHKPSNTKVDKRVESKYGPPCPPCPAPEFLGGPSVFLFPPKPKDTLMISRTPEVTCVVVDVSQEDPEVQFNWYVDGVEVHNAKTKPREEQFNSTYRVVSVLTVLHQDWLNGKEYKCKVSNKGLPSSIEKTISKAKGQPREPQVYTLPPSQEEMTKNQVSLTCLVKGFYPSDIAVEWESNGQPENNYKTTPPVLDSDGSFFLYSRLTVDKSRWQEGNVFSCSVMHEALHNHYTQKSLSLSLGK

SEQ ID NO: 49 - DNA, 1341 bp, Artificial Sequence
  source: /note="Description of Artificial Sequence: Synthetic polynucleotide"
gaggtccagctggtacagtctggggctgaggtgaagaagcctggggctacagtgaaaatctcctgcaaggtttctggctacaccttcaccagttactggatgtactggatcaggcagtccccatcgagaggccttgagtggctgggtaggattgatcctaatagtgggagtactaagtacaatgagaagttcaagaacagactcaccatctccaaggacacctccaaaaaccaggtggtccttacaatgaccaacatggaccctgtggacacagccacgtattactgtgcaagggactatagaaaggggctctatgctatggactactggggccagggcaccaccgtgaccgtgtcctccgcttccaccaagggcccatccgtcttccccctggcgccctgctccaggagcacctccgagagcacagccgccctgggctgcctggtcaaggactacttccccgaaccggtgacggtgtcgtggaactcaggcgccctgaccagcggcgtgcacaccttcccggctgtcctacagtcctcaggactctactccctcagcagcgtggtgaccgtgccctccagcagcttgggcacgaagacctacacctgcaacgtagatcacaagcccagcaacaccaaggtggacaagagagttgagtccaaatatggtcccccatgcccaccgtgcccagcacctgagttcctggggggaccatcagtcttcctgttccccccaaaacccaaggacactctcatgatctcccggacccctgaggtcacgtgcgtggtggtggacgtgagccaggaagaccccgaggtccagttcaactggtacgtggatggcgtggaggtgcataatgccaagacaaagccgcgggaggagcagttcaacagcacgtaccgtgtggtcagcgtcctcaccgtcctgcaccaggactggctgaacggcaaggagtacaagtgcaaggtgtccaacaaaggcctcccgtcctccatcgagaaaaccatctccaaagccaaagggcagccccgagagccacaggtgtacaccctgcccccatcccaggaggagatgaccaagaaccaggtcagcctgacctgcctggtcaaaggcttctaccccagcgacatcgccgtggagtgggagagcaatgggcagccggagaacaactacaagaccacgcctcccgtgctggactccgacggctccttcttcctctacagcaggctaaccgtggacaagagcaggtggcaggaggggaatgtcttctcatgctccgtgatgcatgaggctctgcacaaccactacacacagaagagcctctccctgtctctgggtaaa

SEQ ID NO: 50 - protein, 120 aa, Artificial Sequence
  source: /note="Description of Artificial Sequence: Synthetic polypeptide"
EVQLVQSGAEVKKPGESLRISCKGSGYTFTSYWMYWIRQPPGKGLEWIGRIDPNSGSTKYNEKFKNRVTITADKSTSTAYMELSSLRSEDTAVYYCARDYRKGLYAMDYWGQGTTVTVSS

SEQ ID NO: 51 - DNA, 360 bp, Artificial Sequence
  source: /note="Description of Artificial Sequence: Synthetic polynucleotide"
gaagtgcagctggtgcagtctggagcagaggtgaaaaagcccggggagtctctgaggatctcctgtaagggttctggctacaccttcaccagttactggatgtactggatccgccagcccccagggaaggggctggagtggattggtaggattgatcctaatagtgggagtactaagtacaatgagaagttcaagaacagagtcacgattaccgcggacaaatccacgagcacagcctacatggagctgagcagcctgagatctgaggacacggccgtgtattactgtgcaagggactatagaaaggggctctatgctatggactactggggccagggcaccaccgtgaccgtgtcctcc

SEQ ID NO: 52 - protein, 447 aa, Artificial Sequence
  source: /note="Description of Artificial Sequence: Synthetic polypeptide"
EVQLVQSGAEVKKPGESLRISCKGSGYTFTSYWMYWIRQPPGKGLEWIGRIDPNSGSTKYNEKFKNRVTITADKSTSTAYMELSSLRSEDTAVYYCARDYRKGLYAMDYWGQGTTVTVSSASTKGPSVFPLAPCSRSTSESTAALGCLVKDYFPEPVTVSWNSGALTSGVHTFPAVLQSSGLYSLSSVVTVPSSSLGTKTYTCNVDHKPSNTKVDKRVESKYGPPCPPCPAPEFLGGPSVFLFPPKPKDTLMISRTPEVTCVVVDVSQEDPEVQFNWYVDGVEVHNAKTKPREEQFNSTYRVVSVLTVLHQDWLNGKEYKCKVSNKGLPSSIEKTISKAKGQPREPQVYTLPPSQEEMTKNQVSLTCLVKGFYPSDIAVEWESNGQPENNYKTTPPVLDSDGSFFLYSRLTVDKSRWQEGNVFSCSVMHEALHNHYTQKSLSLSLGK

SEQ ID NO: 53 - DNA, 1341 bp, Artificial Sequence
  source: /note="Description of Artificial Sequence: Synthetic polynucleotide"
gaagtgcagctggtgcagtctggagcagaggtgaaaaagcccggggagtctctgaggatctcctgtaagggttctggctacaccttcaccagttactggatgtactggatccgccagcccccagggaaggggctggagtggattggtaggattgatcctaatagtgggagtactaagtacaatgagaagttcaagaacagagtcacgattaccgcggacaaatccacgagcacagcctacatggagctgagcagcctgagatctgaggacacggccgtgtattactgtgcaagggactatagaaaggggctctatgctatggactactggggccagggcaccaccgtgaccgtgtcctccgcttccaccaagggcccatccgtcttccccctggcgccctgctccaggagcacctccgagagcacagccgccctgggctgcctggtcaaggactacttccccgaaccggtgacggtgtcgtggaactcaggcgccctgaccagcggcgtgcacaccttcccggctgtcctacagtcctcaggactctactccctcagcagcgtggtgaccgtgccctccagcagcttgggcacgaagacctacacctgcaacgtagatcacaagcccagcaacaccaaggtggacaagagagttgagtccaaatatggtcccccatgcccaccgtgcccagcacctgagttcctggggggaccatcagtcttcctgttccccccaaaacccaaggacactctcatgatctcccggacccctgaggtcacgtgcgtggtggtggacgtgagccaggaagaccccgaggtccagttcaactggtacgtggatggcgtggaggtgcataatgccaagacaaagccgcgggaggagcagttcaacagcacgtaccgtgtggtcagcgtcctcaccgtcctgcaccaggactggctgaacggcaaggagtacaagtgcaaggtgtccaacaaaggcctcccgtcctccatcgagaaaaccatctccaaagccaaagggcagccccgagagccacaggtgtacaccctgcccccatcccaggaggagatgaccaagaaccaggtcagcctgacctgcctggtcaaaggcttctaccccagcgacatcgccgtggagtgggagagcaatgggcagccggagaacaactacaagaccacgcctcccgtgctggactccgacggctccttcttcctctacagcaggctaaccgtggacaagagcaggtggcaggaggggaatgtcttctcatgctccgtgatgcatgaggctctgcacaaccactacacacagaagagcctctccctgtctctgggtaaa

SEQ ID NO: 54 - protein, 120 aa, Artificial Sequence
  source: /note="Description of Artificial Sequence: Synthetic polypeptide"
QVQLVQSGAEVKKPGASVKVSCKASGYTFTSYWMYWIRQSPSRGLEWLGRIDPNSGSTKYNEKFKNRFTISRDDSKNTAYLQMNSLKTEDTAVYYCARDYRKGLYAMDYWGQGTTVTVSS

SEQ ID NO: 55 - DNA, 360 bp, Artificial Sequence
  source: /note="Description of Artificial Sequence: Synthetic polynucleotide"
caggttcagctggtgcagtctggagctgaggtgaagaagcctggggcctcagtgaaggtctcctgcaaggcttctggctacaccttcaccagttactggatgtactggatcaggcagtccccatcgagaggccttgagtggctgggtaggattgatcctaatagtgggagtactaagtacaatgagaagttcaagaacagattcaccatctccagagatgattcaaagaacacggcgtatctgcaaatgaacagcctgaaaaccgaggacacggccgtgtattactgtgcaagggactatagaaaggggctctatgctatggactactggggccagggcaccaccgtgaccgtgtcctcc

SEQ ID NO: 56 - protein, 447 aa, Artificial Sequence
  source: /note="Description of Artificial Sequence: Synthetic polypeptide"
QVQLVQSGAEVKKPGASVKVSCKASGYTFTSYWMYWIRQSPSRGLEWLGRIDPNSGSTKYNEKFKNRFTISRDDSKNTAYLQMNSLKTEDTAVYYCARDYRKGLYAMDYWGQGTTVTVSSASTKGPSVFPLAPCSRSTSESTAALGCLVKDYFPEPVTVSWNSGALTSGVHTFPAVLQSSGLYSLSSVVTVPSSSLGTKTYTCNVDHKPSNTKVDKRVESKYGPPCPPCPAPEFLGGPSVFLFPPKPKDTLMISRTPEVTCVVVDVSQEDPEVQFNWYVDGVEVHNAKTKPREEQFNSTYRVVSVLTVLHQDWLNGKEYKCKVSNKGLPSSIEKTISKAKGQPREPQVYTLPPSQEEMTKNQVSLTCLVKGFYPSDIAVEWESNGQPENNYKTTPPVLDSDGSFFLYSRLTVDKSRWQEGNVFSCSVMHEALHNHYTQKSLSLSLGK

SEQ ID NO: 57 - DNA, 1341 bp, Artificial Sequence
  source: /note="Description of Artificial Sequence: Synthetic polynucleotide"
caggttcagctggtgcagtctggagctgaggtgaagaagcctggggcctcagtgaaggtctcctgcaaggcttctggctacaccttcaccagttactggatgtactggatcaggcagtccccatcgagaggccttgagtggctgggtaggattgatcctaatagtgggagtactaagtacaatgagaagttcaagaacagattcaccatctccagagatgattcaaagaacacggcgtatctgcaaatgaacagcctgaaaaccgaggacacggccgtgtattactgtgcaagggactatagaaaggggctctatgctatggactactggggccagggcaccaccgtgaccgtgtcctccgcttccaccaagggcccatccgtcttccccctggcgccctgctccaggagcacctccgagagcacagccgccctgggctgcctggtcaaggactacttccccgaaccggtgacggtgtcgtggaactcaggcgccctgaccagcggcgtgcacaccttcccggctgtcctacagtcctcaggactctactccctcagcagcgtggtgaccgtgccctccagcagcttgggcacgaagacctacacctgcaacgtagatcacaagcccagcaacaccaaggtggacaagagagttgagtccaaatatggtcccccatgcccaccgtgcccagcacctgagttcctggggggaccatcagtcttcctgttccccccaaaacccaaggacactctcatgatctcccggacccctgaggtcacgtgcgtggtggtggacgtgagccaggaagaccccgaggtccagttcaactggtacgtggatggcgtggaggtgcataatgccaagacaaagccgcgggaggagcagttcaacagcacgtaccgtgtggtcagcgtcctcaccgtcctgcaccaggactggctgaacggcaaggagtacaagtgcaaggtgtccaacaaaggcctcccgtcctccatcgagaaaaccatctccaaagccaaagggcagccccgagagccacaggtgtacaccctgcccccatcccaggaggagatgaccaagaaccaggtcagcctgacctgcctggtcaaaggcttctaccccagcgacatcgccgtggagtgggagagcaatgggcagccggagaacaactacaagaccacgcctcccgtgctggactccgacggctccttcttcctctacagcaggctaaccgtggacaagagcaggtggcaggaggggaatgtcttctcatgctccgtgatgcatgaggctctgcacaaccactacacacagaagagcctctccctgtctctgggtaaa

SEQ ID NO: 58 - protein, 107 aa, Artificial Sequence
  source: /note="Description of Artificial Sequence: Synthetic polypeptide"
EIVLTQSPATLSLSPGERATLSCKASQDVGTAVAWYLQKPGQSPQLLIYWASTRHTGIPPRFSGSGYGTDFTLTINNIESEDAAYYFCQQYNSYPLTFGQGTKVEIK

SEQ ID NO: 59 - DNA, 321 bp, Artificial Sequence
  source: /note="Description of Artificial Sequence: Synthetic polynucleotide"
gaaattgtgttgacacagtctccagccaccctgtctttgtctccaggggaaagagccaccctctcctgcaaggccagtcaggatgtgggtactgctgtagcctggtacctgcagaagccagggcagtctccacagctcctgatctattgggcatccacccggcacactgggatcccacctcgattcagtggcagcgggtatggaacagattttaccctcacaattaataacatagaatctgaggatgctgcatattacttctgtcagcagtataacagctatcctctcacgttcggccaagggaccaaggtggaaatcaaa

SEQ ID NO: 60 - protein, 214 aa, Artificial Sequence
  source: /note="Description of Artificial Sequence: Synthetic polypeptide"
EIVLTQSPATLSLSPGERATLSCKASQDVGTAVAWYLQKPGQSPQLLIYWASTRHTGIPPRFSGSGYGTDFTLTINNIESEDAAYYFCQQYNSYPLTFGQGTKVEIKRTVAAPSVFIFPPSDEQLKSGTASVVCLLNNFYPREAKVQWKVDNALQSGNSQESVTEQDSKDSTYSLSSTLTLSKADYEKHKVYACEVTHQGLSSPVTKSFNRGEC

SEQ ID NO: 61 - DNA, 642 bp, Artificial Sequence
  source: /note="Description of Artificial Sequence: Synthetic polynucleotide"
gaaattgtgttgacacagtctccagccaccctgtctttgtctccaggggaaagagccaccctctcctgcaaggccagtcaggatgtgggtactgctgtagcctggtacctgcagaagccagggcagtctccacagctcctgatctattgggcatccacccggcacactgggatcccacctcgattcagtggcagcgggtatggaacagattttaccctcacaattaataacatagaatctgaggatgctgcatattacttctgtcagcagtataacagctatcctctcacgttcggccaagggaccaaggtggaaatcaaacgtacggtggctgcaccatctgtcttcatcttcccgccatctgatgagcagttgaaatctggaactgcctctgttgtgtgcctgctgaataacttctatcccagagaggccaaagtacagtggaaggtggataacgccctccaatcgggtaactcccaggagagtgtcacagagcaggacagcaaggacagcacctacagcctcagcagcaccctgacgctgagcaaagcagactacgagaaacacaaagtctacgcctgcgaagtcacccatcagggcctgagctcgcccgtcacaaagagcttcaacaggggagagtgt

SEQ ID NO: 62 - protein, 120 aa, Artificial Sequence
  source: /note="Description of Artificial Sequence: Synthetic polypeptide"
EVQLVQSGAEVKKPGESLRISCKGSGYTFTSYWMYWVRQARGQRLEWIGRIDPNSGSTKYNEKFKNRLTISKDTSKNQVVLTMTNMDPVDTATYYCARDYRKGLYAMDYWGQGTTVTVSS

SEQ ID NO: 63 - DNA, 360 bp, Artificial Sequence
  source: /note="Description of Artificial Sequence: Synthetic polynucleotide"
gaagtgcagctggtgcagtctggagcagaggtgaaaaagcccggggagtctctgaggatctcctgtaagggttctggctacaccttcaccagttactggatgtactgggtgcgacaggctcgtggacaacgccttgagtggataggtaggattgatcctaatagtgggagtactaagtacaatgagaagttcaagaacagactcaccatctccaaggacacctccaaaaaccaggtggtccttacaatgaccaacatggaccctgtggacacagccacgtattactgtgcaagggactatagaaaggggctctatgctatggactactggggccagggcaccaccgtgaccgtgtcctcc

SEQ ID NO: 64 - protein, 447 aa, Artificial Sequence
  source: /note="Description of Artificial Sequence: Synthetic polypeptide"
EVQLVQSGAEVKKPGESLRISCKGSGYTFTSYWMYWVRQARGQRLEWIGRIDPNSGSTKYNEKFKNRLTISKDTSKNQVVLTMTNMDPVDTATYYCARDYRKGLYAMDYWGQGTTVTVSSASTKGPSVFPLAPCSRSTSESTAALGCLVKDYFPEPVTVSWNSGALTSGVHTFPAVLQSSGLYSLSSVVTVPSSSLGTKTYTCNVDHKPSNTKVDKRVESKYGPPCPPCPAPEFLGGPSVFLFPPKPKDTLMISRTPEVTCVVVDVSQEDPEVQFNWYVDGVEVHNAKTKPREEQFNSTYRVVSVLTVLHQDWLNGKEYKCKVSNKGLPSSIEKTISKAKGQPREPQVYTLPPSQEEMTKNQVSLTCLVKGFYPSDIAVEWESNGQPENNYKTTPPVLDSDGSFFLYSRLTVDKSRWQEGNVFSCSVMHEALHNHYTQKSLSLSLGK

SEQ ID NO: 65 - DNA, 1341 bp, Artificial Sequence
  source: /note="Description of Artificial Sequence: Synthetic polynucleotide"
gaagtgcagctggtgcagtctggagcagaggtgaaaaagcccggggagtctctgaggatctcctgtaagggttctggctacaccttcaccagttactggatgtactgggtgcgacaggctcgtggacaacgccttgagtggataggtaggattgatcctaatagtgggagtactaagtacaatgagaagttcaagaacagactcaccatctccaaggacacctccaaaaaccaggtggtccttacaatgaccaacatggaccctgtggacacagccacgtattactgtgcaagggactatagaaaggggctctatgctatggactactggggccagggcaccaccgtgaccgtgtcctccgcttccaccaagggcccatccgtcttccccctggcgccctgctccaggagcacctccgagagcacagccgccctgggctgcctggtcaaggactacttccccgaaccggtgacggtgtcgtggaactcaggcgccctgaccagcggcgtgcacaccttcccggctgtcctacagtcctcaggactctactccctcagcagcgtggtgaccgtgccctccagcagcttgggcacgaagacctacacctgcaacgtagatcacaagcccagcaacaccaaggtggacaagagagttgagtccaaatatggtcccccatgcccaccgtgcccagcacctgagttcctggggggaccatcagtcttcctgttccccccaaaacccaaggacactctcatgatctcccggacccctgaggtcacgtgcgtggtggtggacgtgagccaggaagaccccgaggtccagttcaactggtacgtggatggcgtggaggtgcataatgccaagacaaagccgcgggaggagcagttcaacagcacgtaccgtgtggtcagcgtcctcaccgtcctgcaccaggactggctgaacggcaaggagtacaagtgcaaggtgtccaacaaaggcctcccgtcctccatcgagaaaaccatctccaaagccaaagggcagccccgagagccacaggtgtacaccctgcccccatcccaggaggagatgaccaagaaccaggtcagcctgacctgcctggtcaaaggcttctaccccagcgacatcgccgtggagtgggagagcaatgggcagccggagaacaactacaagaccacgcctcccgtgctggactccgacggctccttcttcctctacagcaggctaaccgtggacaagagcaggtggcaggaggggaatgtcttctcatgctccgtgatgcatgaggctctgcacaaccactacacacagaagagcctctccctgtctctgggtaaa

SEQ ID NO: 66 - protein, 107 aa, Artificial Sequence
  source: /note="Description of Artificial Sequence: Synthetic polypeptide"
DVVMTQSPLSLPVTLGQPASISCKASQDVGTAVAWYQQKPGQAPRLLIYWASTRHTGVPSRFSGSGSGTEFTLTISSLQPDDFATYYCQQYNSYPLTFGQGTKVEIK

SEQ ID NO: 67 - DNA, 321 bp, Artificial Sequence
  source: /note="Description of Artificial Sequence: Synthetic polynucleotide"
gatgttgtgatgactcagtctccactctccctgcccgtcacccttggacagccggcctccatctcctgcaaggccagtcaggatgtgggtactgctgtagcctggtaccagcagaaacctggccaggctcccaggctcctcatctattgggcatccacccggcacactggggtcccatcaaggttcagcggcagtggatctgggacagaattcactctcaccatcagcagcctgcagcctgatgattttgcaacttattactgtcagcagtataacagctatcctctcacgttcggccaagggaccaaggtggaaatcaaa

SEQ ID NO: 68 - protein, 214 aa, Artificial Sequence
  source: /note="Description of Artificial Sequence: Synthetic polypeptide"
DVVMTQSPLSLPVTLGQPASISCKASQDVGTAVAWYQQKPGQAPRLLIYWASTRHTGVPSRFSGSGSGTEFTLTISSLQPDDFATYYCQQYNSYPLTFGQGTKVEIKRTVAAPSVFIFPPSDEQLKSGTASVVCLLNNFYPREAKVQWKVDNALQSGNSQESVTEQDSKDSTYSLSSTLTLSKADYEKHKVYACEVTHQGLSSPVTKSFNRGEC

SEQ ID NO: 69 - DNA, 642 bp, Artificial Sequence
  source: /note="Description of Artificial Sequence: Synthetic polynucleotide"
gatgttgtgatgactcagtctccactctccctgcccgtcacccttggacagccggcctccatctcctgcaaggccagtcaggatgtgggtactgctgtagcctggtaccagcagaaacctggccaggctcccaggctcctcatctattgggcatccacccggcacactggggtcccatcaaggttcagcggcagtggatctgggacagaattcactctcaccatcagcagcctgcagcctgatgattttgcaacttattactgtcagcagtataacagctatcctctcacgttcggccaagggaccaaggtggaaatcaaacgtacggtggctgcaccatctgtcttcatcttcccgccatctgatgagcagttgaaatctggaactgcctctgttgtgtgcctgctgaataacttctatcccagagaggccaaagtacagtggaaggtggataacgccctccaatcgggtaactcccaggagagtgtcacagagcaggacagcaaggacagcacctacagcctcagcagcaccctgacgctgagcaaagcagactacgagaaacacaaagtctacgcctgcgaagtcacccatcagggcctgagctcgcccgtcacaaagagcttcaacaggggagagtgt

SEQ ID NO: 70 - protein, 120 aa, Artificial Sequence
  source: /note="Description of Artificial Sequence: Synthetic polypeptide"
QITLKESGPTLVKPTQTLTLTCTFSGYTFTSYWMYWVRQAPGKGLEWVSRIDPNSGSTKYNEKFKNRVTITADKSTSTAYMELSSLRSEDTAVYYCARDYRKGLYAMDYWGQGTTVTVSS

SEQ ID NO: 71 - DNA, 360 bp, Artificial Sequence
  source: /note="Description of Artificial Sequence: Synthetic polynucleotide"
cagatcaccttgaaggagtctggtcctacgctggtgaaacccacacagaccctcacgctgacctgcaccttctctggctacaccttcaccagttactggatgtactgggtccgccaggctccagggaaggggctggagtgggtcagtaggattgatcctaatagtgggagtactaagtacaatgagaagttcaagaacagagtcacgattaccgcggacaaatccacgagcacagcctacatggagctgagcagcctgagatctgaggacacggccgtgtattactgtgcaagggactatagaaaggggctctatgctatggactactggggccagggcaccaccgtgaccgtgtcctcc

SEQ ID NO: 72 - protein, 447 aa, Artificial Sequence
  source: /note="Description of Artificial Sequence: Synthetic polypeptide"
QITLKESGPTLVKPTQTLTLTCTFSGYTFTSYWMYWVRQAPGKGLEWVSRIDPNSGSTKYNEKFKNRVTITADKSTSTAYMELSSLRSEDTAVYYCARDYRKGLYAMDYWGQGTTVTVSSASTKGPSVFPLAPCSRSTSESTAALGCLVKDYFPEPVTVSWNSGALTSGVHTFPAVLQSSGLYSLSSVVTVPSSSLGTKTYTCNVDHKPSNTKVDKRVESKYGPPCPPCPAPEFLGGPSVFLFPPKPKDTLMISRTPEVTCVVVDVSQEDPEVQFNWYVDGVEVHNAKTKPREEQFNSTYRVVSVLTVLHQDWLNGKEYKCKVSNKGLPSSIEKTISKAKGQPREPQVYTLPPSQEEMTKNQVSLTCLVKGFYPSDIAVEWESNGQPENNYKTTPPVLDSDGSFFLYSRLTVDKSRWQEGNVFSCSVMHEALHNHYTQKSLSLSLGK

SEQ ID NO: 73 - DNA, 1341 bp, Artificial Sequence
  source: /note="Description of Artificial Sequence: Synthetic polynucleotide"
cagatcaccttgaaggagtctggtcctacgctggtgaaacccacacagaccctcacgctgacctgcaccttctctggctacaccttcaccagttactggatgtactgggtccgccaggctccagggaaggggctggagtgggtcagtaggattgatcctaatagtgggagtactaagtacaatgagaagttcaagaacagagtcacgattaccgcggacaaatccacgagcacagcctacatggagctgagcagcctgagatctgaggacacggccgtgtattactgtgcaagggactatagaaaggggctctatgctatggactactggggccagggcaccaccgtgaccgtgtcctccgcttccaccaagggcccatccgtcttccccctggcgccctgctccaggagcacctccgagagcacagccgccctgggctgcctggtcaaggactacttccccgaaccggtgacggtgtcgtggaactcaggcgccctgaccagcggcgtgcacaccttcccggctgtcctacagtcctcaggactctactccctcagcagcgtggtgaccgtgccctccagcagcttgggcacgaagacctacacctgcaacgtagatcacaagcccagcaacaccaaggtggacaagagagttgagtccaaatatggtcccccatgcccaccgtgcccagcacctgagttcctggggggaccatcagtcttcctgttccccccaaaacccaaggacactctcatgatctcccggacccctgaggtcacgtgcgtggtggtggacgtgagccaggaagaccccgaggtccagttcaactggtacgtggatggcgtggaggtgcataatgccaagacaaagccgcgggaggagcagttcaacagcacgtaccgtgtggtcagcgtcctcaccgtcctgcaccaggactggctgaacggcaaggagtacaagtgcaaggtgtccaacaaaggcctcccgtcctccatcgagaaaaccatctccaaagccaaagggcagccccgagagccacaggtgtacaccctgcccccatcccaggaggagatgaccaagaaccaggtcagcctgacctgcctggtcaaaggcttctaccccagcgacatcgccgtggagtgggagagcaatgggcagccggagaacaactacaagaccacgcctcccgtgctggactccgacggctccttcttcctctacagcaggctaaccgtggacaagagcaggtggcaggaggggaatgtcttctcatgctccgtgatgcatgaggctctgcacaaccactacacacagaagagcctctccctgtctctgggtaaa

SEQ ID NO: 74 - protein, 107 aa, Artificial Sequence
  source: /note="Description of Artificial Sequence: Synthetic polypeptide"
DIQMTQSPSSLSASVGDRVTITCKASQDVGTAVAWYQQKPGQAPRLLIYWASTRHTGVPSRFSGSGSGTDFTFTISSLQPEDIATYYCQQYNSYPLTFGQGTKVEIK

SEQ ID NO: 75 - DNA, 321 bp, Artificial Sequence
  source: /note="Description of Artificial Sequence: Synthetic polynucleotide"
gacatccagatgacccagtctccatcctccctgtctgcatctgtaggagacagagtcaccatcacttgcaaggccagtcaggatgtgggtactgctgtagcctggtaccagcagaaacctggccaggctcccaggctcctcatctattgggcatccacccggcacactggggtcccatcaaggttcagtggaagtggatctgggacagattttactttcaccatcagcagcctgcagcctgaagatattgcaacatattactgtcagcagtataacagctatcctctcacgttcggccaagggaccaaggtggaaatcaaa

SEQ ID NO: 76 - protein, 214 aa, Artificial Sequence
  source: /note="Description of Artificial Sequence: Synthetic polypeptide"
DIQMTQSPSSLSASVGDRVTITCKASQDVGTAVAWYQQKPGQAPRLLIYWASTRHTGVPSRFSGSGSGTDFTFTISSLQPEDIATYYCQQYNSYPLTFGQGTKVEIKRTVAAPSVFIFPPSDEQLKSGTASVVCLLNNFYPREAKVQWKVDNALQSGNSQESVTEQDSKDSTYSLSSTLTLSKADYEKHKVYACEVTHQGLSSPVTKSFNRGEC

SEQ ID NO: 77 - DNA, 642 bp, Artificial Sequence
  source: /note="Description of Artificial Sequence: Synthetic polynucleotide"
gacatccagatgacccagtctccatcctccctgtctgcatctgtaggagacagagtcaccatcacttgcaaggccagtcaggatgtgggtactgctgtagcctggtaccagcagaaacctggccaggctcccaggctcctcatctattgggcatccacccggcacactggggtcccatcaaggttcagtggaagtggatctgggacagattttactttcaccatcagcagcctgcagcctgaagatattgcaacatattactgtcagcagtataacagctatcctctcacgttcggccaagggaccaaggtggaaatcaaacgtacggtggctgcaccatctgtcttcatcttcccgccatctgatgagcagttgaaatctggaactgcctctgttgtgtgcctgctgaataacttctatcccagagaggccaaagtacagtggaaggtggataacgccctccaatcgggtaactcccaggagagtgtcacagagcaggacagcaaggacagcacctacagcctcagcagcaccctgacgctgagcaaagcagactacgagaaacacaaagtctacgcctgcgaagtcacccatcagggcctgagctcgcccgtcacaaagagcttcaacaggggagagtgt

SEQ ID NO: 78 - protein, 120 aa, Artificial Sequence
  source: /note="Description of Artificial Sequence: Synthetic polypeptide"
EVQLVQSGAEVKKPGATVKISCKVSGYTFTSYWMYWVRQARGQRLEWIGRIDPNSGSTKYNEKFKNRFTISRDNSKNTLYLQMNSLRAEDTAVYYCARDYRKGLYAMDYWGQGTTVTVSS

SEQ ID NO: 79 - DNA, 360 bp, Artificial Sequence
  source: /note="Description of Artificial Sequence: Synthetic polynucleotide"
gaggtccagctggtacagtctggggctgaggtgaagaagcctggggctacagtgaaaatctcctgcaaggtttctggctacaccttcaccagttactggatgtactgggtgcgacaggctcgtggacaacgccttgagtggataggtaggattgatcctaatagtgggagtactaagtacaatgagaagttcaagaacagattcaccatctccagagacaattccaagaacacgctgtatcttcaaatgaacagcctgagagccgaggacacggccgtgtattactgtgcaagggactatagaaaggggctctatgctatggactactggggccagggcaccaccgtgaccgtgtcctcc

SEQ ID NO: 80 - protein, 446 aa, Artificial Sequence
  source: /note="Description of Artificial Sequence: Synthetic polypeptide"
EVQLVQSGAEVKKPGATVKISCKVSGYTFTSYWMYWVRQARGQRLEWIGRIDPNSGSTKYNEKFKNRFTISRDNSKNTLYLQMNSLRAEDTAVYYCARDYRKGLYAMDYWGQGTTVTVSSASTKGPSVFPLAPCSRSTSESTAALGCLVKDYFPEPVTVSWNSGALTSGVHTFPAVLQSSGLYSLSSVVTVPSSSLGTKTYTCNVDHKPSNTKVDKRVESKYGPPCPPCPAPEFLGGPSVFLFPPKPKDTLMISRTPEVTCVVVDVSQEDPEVQFNWYVDGVEVHNAKTKPREEQFNSTYRVVSVLTVLHQDWLNGKEYKCKVSNKGLPSSIEKTISKAKGQPREPQVYTLPPSQEEMTKNQVSLTCLVKGFYPSDIAVEWESNGQPENNYKTTPPVLDSDGSFFLYSRLTVDKSRWQEGNVFSCSVMHEALHNHYTQKSLSLSLG

SEQ ID NO: 81 - DNA, 1341 bp, Artificial Sequence
  source: /note="Description of Artificial Sequence: Synthetic polynucleotide"
gaggtccagctggtacagtctggggctgaggtgaagaagcctggggctacagtgaaaatctcctgcaaggtttctggctacaccttcaccagttactggatgtactgggtgcgacaggctcgtggacaacgccttgagtggataggtaggattgatcctaatagtgggagtactaagtacaatgagaagttcaagaacagattcaccatctccagagacaattccaagaacacgctgtatcttcaaatgaacagcctgagagccgaggacacggccgtgtattactgtgcaagggactatagaaaggggctctatgctatggactactggggccagggcaccaccgtgaccgtgtcctccgcttccaccaagggcccatccgtcttccccctggcgccctgctccaggagcacctccgagagcacagccgccctgggctgcctggtcaaggactacttccccgaaccggtgacggtgtcgtggaactcaggcgccctgaccagcggcgtgcacaccttcccggctgtcctacagtcctcaggactctactccctcagcagcgtggtgaccgtgccctccagcagcttgggcacgaagacctacacctgcaacgtagatcacaagcccagcaacaccaaggtggacaagagagttgagtccaaatatggtcccccatgcccaccgtgcccagcacctgagttcctggggggaccatcagtcttcctgttccccccaaaacccaaggacactctcatgatctcccggacccctgaggtcacgtgcgtggtggtggacgtgagccaggaagaccccgaggtccagttcaactggtacgtggatggcgtggaggtgcataatgccaagacaaagccgcgggaggagcagttcaacagcacgtaccgtgtggtcagcgtcctcaccgtcctgcaccaggactggctgaacggcaaggagtacaagtgcaaggtgtccaacaaaggcctcccgtcctccatcgagaaaaccatctccaaagccaaagggcagccccgagagccacaggtgtacaccctgcccccatcccaggaggagatgaccaagaaccaggtcagcctgacctgcctggtcaaaggcttctaccccagcgacatcgccgtggagtgggagagcaatgggcagccggagaacaactacaagaccacgcctcccgtgctggactccgacggctccttcttcctctacagcaggctaaccgtggacaagagcaggtggcaggaggggaatgtcttctcatgctccgtgatgcatgaggctctgcacaaccactacacacagaagagcctctccctgtctctgggtaaa

SEQ ID NO: 82 - protein, 107 aa, Artificial Sequence
  source: /note="Description of Artificial Sequence: Synthetic polypeptide"
AIQLTQSPSSLSASVGDRVTITCKASQDVGTAVAWYLQKPGQSPQLLIYWASTRHTGVPSRFSGSGSGTDFTFTISSLEAEDAATYYCQQYNSYPLTFGQGTKVEIK

SEQ ID NO: 83 - DNA, 321 bp, Artificial Sequence
  source: /note="Description of Artificial Sequence: Synthetic polynucleotide"
gccatccagttgacccagtctccatcctccctgtctgcatctgtaggagacagagtcaccatcacttgcaaggccagtcaggatgtgggtactgctgtagcctggtacctgcagaagccagggcagtctccacagctcctgatctattgggcatccacccggcacactggggtcccctcgaggttcagtggcagtggatctgggacagatttcacctttaccatcagtagcctggaagctgaagatgctgcaacatattactgtcagcagtataacagctatcctctcacgttcggccaagggaccaaggtggaaatcaaa

SEQ ID NO: 84 - protein, 214 aa, Artificial Sequence
  source: /note="Description of Artificial Sequence: Synthetic polypeptide"
AIQLTQSPSSLSASVGDRVTITCKASQDVGTAVAWYLQKPGQSPQLLIYWASTRHTGVPSRFSGSGSGTDFTFTISSLEAEDAATYYCQQYNSYPLTFGQGTKVEIKRTVAAPSVFIFPPSDEQLKSGTASVVCLLNNFYPREAKVQWKVDNALQSGNSQESVTEQDSKDSTYSLSSTLTLSKADYEKHKVYACEVTHQGLSSPVTKSFNRGEC

SEQ ID NO: 85 - DNA, 642 bp, Artificial Sequence
  source: /note="Description of Artificial Sequence: Synthetic polynucleotide"
gccatccagttgacccagtctccatcctccctgtctgcatctgtaggagacagagtcaccatcacttgcaaggccagtcaggatgtgggtactgctgtagcctggtacctgcagaagccagggcagtctccacagctcctgatctattgggcatccacccggcacactggggtcccctcgaggttcagtggcagtggatctgggacagatttcacctttaccatcagtagcctggaagctgaagatgctgcaacatattactgtcagcagtataacagctatcctctcacgttcggccaagggaccaaggtggaaatcaaacgtacggtggctgcaccatctgtcttcatcttcccgccatctgatgagcagttgaaatctggaactgcctctgttgtgtgcctgctgaataacttctatcccagagaggccaaagtacagtggaaggtggataacgccctccaatcgggtaactcccaggagagtgtcacagagcaggacagcaaggacagcacctacagcctcagcagcaccctgacgctgagcaaagcagactacgagaaacacaaagtctacgcctgcgaagtcacccatcagggcctgagctcgcccgtcacaaagagcttcaacaggggagagtgt

SEQ ID NO: 86 - protein, 107 aa, Artificial Sequence
  source: /note="Description of Artificial Sequence: Synthetic polypeptide"
EIVLTQSPDFQSVTPKEKVTITCKASQDVGTAVAWYQQKPGQAPRLLIYWASTRHTGVPSRFSGSGSGTEFTLTISSLQPDDFATYYCQQYNSYPLTFGQGTKVEIK

SEQ ID NO: 87 - DNA, 321 bp, Artificial Sequence
  source: /note="Description of Artificial Sequence: Synthetic polynucleotide"
gaaattgtgctgactcagtctccagactttcagtctgtgactccaaaggagaaagtcaccatcacctgcaaggccagtcaggatgtgggtactgctgtagcctggtaccagcagaaacctggccaggctcccaggctcctcatctattgggcatccacccggcacactggggtcccatcaaggttcagcggcagtggatctgggacagaattcactctcaccatcagcagcctgcagcctgatgattttgcaacttattactgtcagcagtataacagctatcctctcacgttcggccaagggaccaaggtggaaatcaaa

SEQ ID NO: 88 - protein, 214 aa, Artificial Sequence
  source: /note="Description of Artificial Sequence: Synthetic polypeptide"
EIVLTQSPDFQSVTPKEKVTITCKASQDVGTAVAWYQQKPGQAPRLLIYWASTRHTGVPSRFSGSGSGTEFTLTISSLQPDDFATYYCQQYNSYPLTFGQGTKVEIKRTVAAPSVFIFPPSDEQLKSGTASVVCLLNNFYPREAKVQWKVDNALQSGNSQESVTEQDSKDSTYSLSSTLTLSKADYEKHKVYACEVTHQGLSSPVTKSFNRGEC

SEQ ID NO: 89 - DNA, 642 bp, Artificial Sequence
  source: /note="Description of Artificial Sequence: Synthetic polynucleotide"
gaaattgtgctgactcagtctccagactttcagtctgtgactccaaaggagaaagtcaccatcacctgcaaggccagtcaggatgtgggtactgctgtagcctggtaccagcagaaacctggccaggctcccaggctcctcatctattgggcatccacccggcacactggggtcccatcaaggttcagcggcagtggatctgggacagaattcactctcaccatcagcagcctgcagcctgatgattttgcaacttattactgtcagcagtataacagctatcctctcacgttcggccaagggaccaaggtggaaatcaaacgtacggtggctgcaccatctgtcttcatcttcccgccatctgatgagcagttgaaatctggaactgcctctgttgtgtgcctgctgaataacttctatcccagagaggccaaagtacagtggaaggtggataacgccctccaatcgggtaactcccaggagagtgtcacagagcaggacagcaaggacagcacctacagcctcagcagcaccctgacgctgagcaaagcagactacgagaaacacaaagtctacgcctgcgaagtcacccatcagggcctgagctcgcccgtcacaaagagcttcaacaggggagagtgt

SEQ ID NO: 90 - DNA, 360 bp, Artificial Sequence
  source: /note="Description of Artificial Sequence: Synthetic polynucleotide"
gaagtgcagctggtgcagtcaggcgccgaagtgaagaagcccggcgagtcactgagaattagctgtaaaggttcaggctacaccttcactagctactggatgtactgggtccgacaggccccagggcaaggcctggagtggatgggtagaatcgaccctaatagcggctctactaagtataacgagaagtttaagaatagagtgactattagcgtggacacctctaagaatcagtttagcctgaagctgtctagcgtgaccgccgctgacaccgccgtctactactgcgctagagactatagaaagggcctgtacgctatggactactggggtcaaggcactaccgtgaccgtgtcttca

SEQ ID NO: 91 - protein, 446 aa, Artificial Sequence
  source: /note="Description of Artificial Sequence: Synthetic polypeptide"
EVQLVQSGAEVKKPGESLRISCKGSGYTFTSYWMYWVRQAPGQGLEWMGRIDPNSGSTKYNEKFKNRVTISVDTSKNQFSLKLSSVTAADTAVYYCARDYRKGLYAMDYWGQGTTVTVSSASTKGPSVFPLAPCSRSTSESTAALGCLVKDYFPEPVTVSWNSGALTSGVHTFPAVLQSSGLYSLSSVVTVPSSSLGTKTYTCNVDHKPSNTKVDKRVESKYGPPCPPCPAPEFLGGPSVFLFPPKPKDTLMISRTPEVTCVVVDVSQEDPEVQFNWYVDGVEVHNAKTKPREEQFNSTYRVVSVLTVLHQDWLNGKEYKCKVSNKGLPSSIEKTISKAKGQPREPQVYTLPPSQEEMTKNQVSLTCLVKGFYPSDIAVEWESNGQPENNYKTTPPVLDSDGSFFLYSRLTVDKSRWQEGNVFSCSVMHEALHNHYTQKSLSLSLG

SEQ ID NO: 92 - DNA, 1338 bp, Artificial Sequence
  source: /note="Description of Artificial Sequence: Synthetic polynucleotide"
gaagtgcagctggtgcagtcaggcgccgaagtgaagaagcccggcgagtcactgagaattagctgtaaaggttcaggctacaccttcactagctactggatgtactgggtccgacaggccccagggcaaggcctggagtggatgggtagaatcgaccctaatagcggctctactaagtataacgagaagtttaagaatagagtgactattagcgtggacacctctaagaatcagtttagcctgaagctgtctagcgtgaccgccgctgacaccgccgtctactactgcgctagagactatagaaagggcctgtacgctatggactactggggtcaaggcactaccgtgaccgtgtcttcagctagcactaagggcccgtccgtgttccccctggcaccttgtagccggagcactagcgaatccaccgctgccctcggctgcctggtcaaggattacttcccggagcccgtgaccgtgtcctggaacagcggagccctgacctccggagtgcacaccttccccgctgtgctgcagagctccgggctgtactcgctgtcgtcggtggtcacggtgccttcatctagcctgggtaccaagacctacacttgcaacgtggaccacaagccttccaacactaaggtggacaagcgcgtcgaatcgaagtacggcccaccgtgcccgccttgtcccgcgccggagttcctcggcggtccctcggtctttctgttcccaccgaagcccaaggacactttgatgatttcccgcacccctgaagtgacatgcgtggtcgtggacgtgtcacaggaagatccggaggtgcagttcaattggtacgtggatggcgtcgaggtgcacaacgccaaaaccaagccgagggaggagcagttcaactccacttaccgcgtcgtgtccgtgctgacggtgctgcatcaggactggctgaacgggaaggagtacaagtgcaaagtgtccaacaagggacttcctagctcaatcgaaaagaccatctcgaaagccaagggacagccccgggaaccccaagtgtataccctgccaccgagccaggaagaaatgactaagaaccaagtctcattgacttgccttgtgaagggcttctacccatcggatatcgccgtggaatgggagtccaacggccagccggaaaacaactacaagaccacccctccggtgctggactcagacggatccttcttcctctactcgcggctgaccgtggataagagcagatggcaggagggaaatgtgttcagctgttctgtgatgcatgaagccctgcacaaccactacactcagaagtccctgtccctctccctggga

SEQ ID NO: 93 - DNA, 321 bp, Artificial Sequence
  source: /note="Description of Artificial Sequence: Synthetic polynucleotide"
gagatcgtcctgactcagtcacccgactttcagtcagtgacccctaaagagaaagtcactatcacctgtaaagcctctcaggacgtgggcaccgccgtggcctggtatctgcagaagcctggtcaatcacctcagctgctgatctactgggcctctactagacacaccggcgtgccctctaggtttagcggtagcggtagtggcaccgacttcaccttcactatctcttcactgcagcccgaggatatcgctacctactactgtcagcagtataatagctaccccctgaccttcggtcaaggcactaaggtcgagattaag

SEQ ID NO: 94 - DNA, 642 bp, Artificial Sequence
  source: /note="Description of Artificial Sequence: Synthetic polynucleotide"
gagatcgtcctgactcagtcacccgactttcagtcagtgacccctaaagagaaagtcactatcacctgtaaagcctctcaggacgtgggcaccgccgtggcctggtatctgcagaagcctggtcaatcacctcagctgctgatctactgggcctctactagacacaccggcgtgccctctaggtttagcggtagcggtagtggcaccgacttcaccttcactatctcttcactgcagcccgaggatatcgctacctactactgtcagcagtataatagctaccccctgaccttcggtcaaggcactaaggtcgagattaagcgtacggtggccgctcccagcgtgttcatcttcccccccagcgacgagcagctgaagagcggcaccgccagcgtggtgtgcctgctgaacaacttctacccccgggaggccaaggtgcagtggaaggtggacaacgccctgcagagcggcaacagccaggagagcgtcaccgagcaggacagcaaggactccacctacagcctgagcagcaccctgaccctgagcaaggccgactacgagaagcataaggtgtacgcctgcgaggtgacccaccagggcctgtccagccccgtgaccaagagcttcaacaggggcgagtgc

SEQ ID NO: 95 - DNA, 360 bp, Artificial Sequence
  source: /note="Description of Artificial Sequence: Synthetic polynucleotide"
gaagtgcagctggtgcagtcaggcgccgaagtgaagaaacccggcgctaccgtgaagattagctgtaaagtctcaggctacaccttcactagctactggatgtactgggtccgacaggctaccggtcaaggcctggagtggatgggtagaatcgaccctaatagcggctctactaagtataacgagaagtttaagaatagagtgactatcaccgccgataagtctactagcaccgcctatatggaactgtctagcctgagatcagaggacaccgccgtctactactgcgctagagactatagaaagggcctgtacgctatggactactggggtcaaggcactaccgtgaccgtgtcttca

SEQ ID NO: 96 - protein, 446 aa, Artificial Sequence
  source: /note="Description of Artificial Sequence: Synthetic polypeptide"
EVQLVQSGAEVKKPGATVKISCKVSGYTFTSYWMYWVRQATGQGLEWMGRIDPNSGSTKYNEKFKNRVTITADKSTSTAYMELSSLRSEDTAVYYCARDYRKGLYAMDYWGQGTTVTVSSASTKGPSVFPLAPCSRSTSESTAALGCLVKDYFPEPVTVSWNSGALTSGVHTFPAVLQSSGLYSLSSVVTVPSSSLGTKTYTCNVDHKPSNTKVDKRVESKYGPPCPPCPAPEFLGGPSVFLFPPKPKDTLMISRTPEVTCVVVDVSQEDPEVQFNWYVDGVEVHNAKTKPREEQFNSTYRVVSVLTVLHQDWLNGKEYKCKVSNKGLPSSIEKTISKAKGQPREPQVYTLPPSQEEMTKNQVSLTCLVKGFYPSDIAVEWESNGQPENNYKTTPPVLDSDGSFFLYSRLTVDKSRWQEGNVFSCSVMHEALHNHYTQKSLSLSLG

SEQ ID NO: 97 - DNA, 1338 bp, Artificial Sequence
  source: /note="Description of Artificial Sequence: Synthetic polynucleotide"
gaagtgcagctggtgcagtcaggcgccgaagtgaagaaacccggcgctaccgtgaagattagctgtaaagtctcaggctacaccttcactagctactggatgtactgggtccgacaggctaccggtcaaggcctggagtggatgggtagaatcgaccctaatagcggctctactaagtataacgagaagtttaagaatagagtgactatcaccgccgataagtctactagcaccgcctatatggaactgtctagcctgagatcagaggacaccgccgtctactactgcgctagagactatagaaagggcctgtacgctatggactactggggtcaaggcactaccgtgaccgtgtcttcagctagcactaagggcccgtccgtgttccccctggcaccttgtagccggagcactagcgaatccaccgctgccctcggctgcctggtcaaggattacttcccggagcccgtgaccgtgtcctggaacagcggagccctgacctccggagtgcacaccttccccgctgtgctgcagagctccgggctgtactcgctgtcgtcggtggtcacggtgccttcatctagcctgggtaccaagacctacacttgcaacgtggaccacaagccttccaacactaaggtggacaagcgcgtcgaatcgaagtacggcccaccgtgcccgccttgtcccgcgccggagttcctcggcggtccctcggtctttctgttcccaccgaagcccaaggacactttgatgatttcccgcacccctgaagtgacatgcgtggtcgtggacgtgtcacaggaagatccggaggtgcagttcaattggtacgtggatggcgtcgaggtgcacaacgccaaaaccaagccgagggaggagcagttcaactccacttaccgcgtcgtgtccgtgctgacggtgctgcatcaggactggctgaacgggaaggagtacaagtgcaaagtgtccaacaagggacttcctagctcaatcgaaaagaccatctcgaaagccaagggacagccccgggaaccccaagtgtataccctgccaccgagccaggaagaaatgactaagaaccaagtctcattgacttgccttgtgaagggcttctacccatcggatatcgccgtggaatgggagtccaacggccagccggaaaacaactacaagaccacccctccggtgctggactcagacggatccttcttcctctactcgcggctgaccgtggataagagcagatggcaggagggaaatgtgttcagctgttctgtgatgcatgaagccctgcacaaccactacactcagaagtccctgtccctctccctggga

SEQ ID NO: 98 - DNA, 321 bp, Artificial Sequence
  source: /note="Description of Artificial Sequence: Synthetic polynucleotide"
gacgtcgtgatgactcagtcacccctgagcctgcccgtgaccctggggcagcccgcctctattagctgtaaagcctctcaggacgtgggcaccgccgtggcctggtatcagcagaagccagggcaagcccctagactgctgatctactgggcctctactagacacaccggcgtgccctctaggtttagcggtagcggtagtggcaccgagttcaccctgactatctcttcactgcagcccgacgacttcgctacctactactgtcagcagtataatagctaccccctgaccttcggtcaaggcactaaggtcgagattaag

SEQ ID NO: 99 - DNA, 642 bp, Artificial Sequence
  source: /note="Description of Artificial Sequence: Synthetic polynucleotide"
gacgtcgtgatgactcagtcacccctgagcctgcccgtgaccctggggcagcccgcctctattagctgtaaagcctctcaggacgtgggcaccgccgtggcctggtatcagcagaagccagggcaagcccctagactgctgatctactgggcctctactagacacaccggcgtgccctctaggtttagcggtagcggtagtggcaccgagttcaccctgactatctcttcactgcagcccgacgacttcgctacctactactgtcagcagtataatagctaccccctgaccttcggtcaaggcactaaggtcgagattaagcgtacggtggccgctcccagcgtgttcatcttcccccccagcgacgagcagctgaagagcggcaccgccagcgtggtgtgcctgctgaacaacttctacccccgggaggccaaggtgcagtggaaggtggacaacgccctgcagagcggcaacagccaggagagcgtcaccgagcaggacagcaaggactccacctacagcctgagcagcaccctgaccctgagcaaggccgactacgagaagcataaggtgtacgcctgcgaggtgacccaccagggcctgtccagccccgtgaccaagagcttcaacaggggcgagtgc

SEQ ID NO: 100 - DNA, 360 bp, Artificial Sequence
  source: /note="Description of Artificial Sequence: Synthetic polynucleotide"
gaagtgcagctggtgcagtcaggcgccgaagtgaagaaacccggcgctaccgtgaagattagctgtaaagtctcaggctacaccttcactagctactggatgtactgggtccgacaggctagagggcaaagactggagtggatcggtagaatcgaccctaatagcggctctactaagtataacgagaagtttaagaataggttcactattagtagggataactctaagaacaccctgtacctgcagatgaatagcctgagagccgaggacaccgccgtctactactgcgctagagactatagaaagggcctgtacgctatggactactggggtcaaggcactaccgtgaccgtgtcttca

SEQ ID NO: 101 - DNA, 1338 bp, Artificial Sequence
  source: /note="Description of Artificial Sequence: Synthetic polynucleotide"
gaagtgcagctggtgcagtcaggcgccgaagtgaagaaacccggcgctaccgtgaagattagctgtaaagtctcaggctacaccttcactagctactggatgtactgggtccgacaggctagagggcaaagactggagtggatcggtagaatcgaccctaatagcggctctactaagtataacgagaagtttaagaataggttcactattagtagggataactctaagaacaccctgtacctgcagatgaatagcctgagagccgaggacaccgccgtctactactgcgctagagactatagaaagggcctgtacgctatggactactggggtcaaggcactaccgtgaccgtgtcttcagctagcactaagggcccgtccgtgttccccctggcaccttgtagccggagcactagcgaatccaccgctgccctcggctgcctggtcaaggattacttcccggagcccgtgaccgtgtcctggaacagcggagccctgacctccggagtgcacaccttccccgctgtgctgcagagctccgggctgtactcgctgtcgtcggtggtcacggtgccttcatctagcctgggtaccaagacctacacttgcaacgtggaccacaagccttccaacactaaggtggacaagcgcgtcgaatcgaagtacggcccaccgtgcccgccttgtcccgcgccggagttcctcggcggtccctcggtctttctgttcccaccgaagcccaaggacactttgatgatttcccgcacccctgaagtgacatgcgtggtcgtggacgtgtcacaggaagatccggaggtgcagttcaattggtacgtggatggcgtcgaggtgcacaacgccaaaaccaagccgagggaggagcagttcaactccacttaccgcgtcgtgtccgtgctgacggtgctgcatcaggactggctgaacgggaaggagtacaagtgcaaagtgtccaacaagggacttcctagctcaatcgaaaagaccatctcgaaagccaagggacagccccgggaaccccaagtgtataccctgccaccgagccaggaagaaatgactaagaaccaagtctcattgacttgccttgtgaagggcttctacccatcggatatcgccgtggaatgggagtccaacggccagccggaaaacaactacaagaccacccctccggtgctggactcagacggatccttcttcctctactcgcggctgaccgtggataagagcagatggcaggagggaaatgtgttcagctgttctgtgatgcatgaagccctgcacaaccactacactcagaagtccctgtccctctccctggga

SEQ ID NO: 102 - DNA, 321 bp, Artificial Sequence
  source: /note="Description of Artificial Sequence: Synthetic polynucleotide"
gctattcagctgactcagtcacctagtagcctgagcgctagtgtgggcgatagagtgactatcacctgtaaagcctctcaggacgtgggcaccgccgtggcctggtatctgcagaagcctggtcaatcacctcagctgctgatctactgggcctctactagacacaccggcgtgccctctaggtttagcggtagcggtagtggcaccgacttcaccttcactatctcttcactggaagccgaggacgccgctacctactactgtcagcagtataatagctaccccctgaccttcggtcaaggcactaaggtcgagattaag

SEQ ID NO: 103 - DNA, 642 bp, Artificial Sequence
  source: /note="Description of Artificial Sequence: Synthetic polynucleotide"
gctattcagctgactcagtcacctagtagcctgagcgctagtgtgggcgatagagtgactatcacctgtaaagcctctcaggacgtgggcaccgccgtggcctggtatctgcagaagcctggtcaatcacctcagctgctgatctactgggcctctactagacacaccggcgtgccctctaggtttagcggtagcggtagtggcaccgacttcaccttcactatctcttcactggaagccgaggacgccgctacctactactgtcagcagtataatagctaccccctgaccttcggtcaaggcactaaggtcgagattaagcgtacggtggccgctcccagcgtgttcatcttcccccccagcgacgagcagctgaagagcggcaccgccagcgtggtgtgcctgctgaacaacttctacccccgggaggccaaggtgcagtggaaggtggacaacgccctgcagagcggcaacagccaggagagcgtcaccgagcaggacagcaaggactccacctacagcctgagcagcaccctgaccctgagcaaggccgactacgagaagcataaggtgtacgcctgcgaggtgacccaccagggcctgtccagccccgtgaccaagagcttcaacaggggcgagtgc

SEQ ID NO: 104 - DNA, 15 bp, Artificial Sequence
  source: /note="Description of Artificial Sequence: Synthetic oligonucleotide"
agttactggatgtac

SEQ ID NO: 105 - DNA, 51 bp, Artificial Sequence
  source: /note="Description of Artificial Sequence: Synthetic oligonucleotide"
aggattgatcctaatagtgggagtactaagtacaatgagaagttcaagaac

SEQ ID NO: 106 - DNA, 33 bp, Artificial Sequence
  source: /note="Description of Artificial Sequence: Synthetic oligonucleotide"
gactatagaaaggggctctatgctatggactac

SEQ ID NO: 107 - DNA, 21 bp, Artificial Sequence
  source: /note="Description of Artificial Sequence: Synthetic oligonucleotide"
ggctacaccttcaccagttac

SEQ ID NO: 108 - DNA, 18 bp, Artificial Sequence
  source: /note="Description of Artificial Sequence: Synthetic oligonucleotide"
gatcctaatagtgggagt

SEQ ID NO: 109 - DNA, 27 bp, Artificial Sequence
  source: /note="Description of Artificial Sequence: Synthetic oligonucleotide"
cagcagtataacagctatcctctcacg

SEQ ID NO: 110 - DNA, 21 bp, Artificial Sequence
  source: /note="Description of Artificial Sequence: Synthetic oligonucleotide"
agtcaggatgtgggtactgct

SEQ ID NO: 111 - DNA, 9 bp, Artificial Sequence
  source: /note="Description of Artificial Sequence: Synthetic oligonucleotide"
tgggcatcc

SEQ ID NO: 112 - DNA, 18 bp, Artificial Sequence
  source: /note="Description of Artificial Sequence: Synthetic oligonucleotide"
tataacagctatcctctc

SEQ ID NO: 113 - DNA, 15 bp, Artificial Sequence
  source: /note="Description of Artificial Sequence: Synthetic oligonucleotide"
agctactggatgtac

SEQ ID NO: 114 - DNA, 51 bp, Artificial Sequence
  source: /note="Description of Artificial Sequence: Synthetic oligonucleotide"
agaatcgaccctaatagcggctctactaagtataacgagaagtttaagaat

SEQ ID NO: 115 - DNA, 33 bp, Artificial Sequence
  source: /note="Description of Artificial Sequence: Synthetic oligonucleotide"
gactatagaaagggcctgtacgctatggactac

SEQ ID NO: 116 - DNA, 21 bp, Artificial Sequence
  source: /note="Description of Artificial Sequence: Synthetic oligonucleotide"
ggctacaccttcactagctac

SEQ ID NO: 117 - DNA, 18 bp, Artificial Sequence
  source: /note="Description of Artificial Sequence: Synthetic oligonucleotide"
gaccctaatagcggctct

SEQ ID NO: 118 - DNA, 33 bp, Artificial Sequence
  source: /note="Description of Artificial Sequence: Synthetic oligonucleotide"
aaagcctctcaggacgtgggcaccgccgtggcc

SEQ ID NO: 119 - DNA, 21 bp, Artificial Sequence
  source: /note="Description of Artificial Sequence: Synthetic oligonucleotide"
tgggcctctactagacacacc

SEQ ID NO: 120 - DNA, 27 bp, Artificial Sequence
  source: /note="Description of Artificial Sequence: Synthetic oligonucleotide"
cagcagtataatagctaccccctgacc

SEQ ID NO: 121 - DNA, 21 bp, Artificial Sequence
  source: /note="Description of Artificial Sequence: Synthetic oligonucleotide"
tctcaggacgtgggcaccgcc

SEQ ID NO: 122 - DNA, 9 bp, Artificial Sequence
  source: /note="Description of Artificial Sequence: Synthetic oligonucleotide"
tgggcctct

SEQ ID NO: 123 - DNA, 18 bp, Artificial Sequence
  source: /note="Description of Artificial Sequence: Synthetic oligonucleotide"
tataatagctaccccctg

SEQ ID NO: 124 - protein, 25 aa, Artificial Sequence [sequence omitted]

SEQ ID NO: 125 - DNA, 75 bp, Artificial Sequence
  source: /note="Description of Artificial Sequence: Synthetic oligonucleotide"
caggttcagctggtgcagtctggagctgaggtgaagaagcctggggcctcagtgaaggtctcctgcaaggcttct

SEQ ID NO: 126 - protein, 25 aa, Artificial Sequence
  source: /note="Description of Artificial Sequence: Synthetic peptide"
EVQLVQSGAEVKKPGESLRISCKGS

SEQ ID NO: 127 - DNA, 75 bp, Artificial Sequence
  source: /note="Description of Artificial Sequence: Synthetic oligonucleotide"
gaagtgcagctggtgcagtctggagcagaggtgaaaaagcccggggagtctctgaggatctcctgtaagggttct

SEQ ID NO: 128 - protein, 25 aa, Artificial Sequence
  source: /note="Description of Artificial Sequence: Synthetic peptide"
EVQLVQSGAEVKKPGATVKISCKVS

SEQ ID NO: 129 - DNA, 75 bp, Artificial Sequence
  source: /note="Description of Artificial Sequence: Synthetic oligonucleotide"
gaggtccagctggtacagtctggggctgaggtgaagaagcctggggctacagtgaaaatctcctgcaaggtttct

SEQ ID NO: 130 - protein, 25 aa, Artificial Sequence
  source: /note="Description of Artificial Sequence: Synthetic peptide"
QITLKESGPTLVKPTQTLTLTCTFS

SEQ ID NO: 131 - DNA, 75 bp, Artificial Sequence
  source: /note="Description of Artificial Sequence: Synthetic oligonucleotide"
cagatcaccttgaaggagtctggtcctacgctggtgaaacccacacagaccctcacgctgacctgcaccttctct

SEQ ID NO: 132 - protein, 14 aa, Artificial Sequence
  source: /note="Description of Artificial Sequence: Synthetic peptide"
WVRQATGQGLEWMG

SEQ ID NO: 133 - DNA, 42 bp, Artificial Sequence
  source: /note="Description of Artificial Sequence: Synthetic oligonucleotide"
tgggtgcgacaggccactggacaagggcttgagtggatgggt

SEQ ID NO: 134 - protein, 14 aa, Artificial Sequence
  source: /note="Description of Artificial Sequence: Synthetic peptide"
WVRQAPGQGLEWMG

SEQ ID NO: 135 - DNA, 42 bp, Artificial Sequence
  source: /note="Description of Artificial Sequence: Synthetic oligonucleotide"
tgggtgcgacaggcccctggacaagggcttgagtggatgggt

SEQ ID NO: 136 - protein, 14 aa, Artificial Sequence
  source: /note="Description of Artificial Sequence: Synthetic peptide"
WIRQPPGKGLEWIG

SEQ ID NO: 137 - DNA, 42 bp, Artificial Sequence
  source: /note="Description of Artificial Sequence: Synthetic oligonucleotide"
tggatccgccagcccccagggaaggggctggagtggattggt

SEQ ID NO: 138 - protein, 14 aa, Artificial Sequence
  source: /note="Description of Artificial Sequence: Synthetic peptide"
WIRQSPSRGLEWLG

SEQ ID NO: 139 - DNA, 42 bp, Artificial Sequence
  source: /note="Description of Artificial Sequence: Synthetic oligonucleotide"
tggatcaggcagtccccatcgagaggccttgagtggctgggt

SEQ ID NO: 140 - protein, 14 aa, Artificial Sequence
  source: /note="Description of Artificial Sequence: Synthetic peptide"
WVRQARGQRLEWIG

SEQ ID NO: 141 - DNA, 42 bp, Artificial Sequence
  source: /note="Description of Artificial Sequence: Synthetic oligonucleotide"
tgggtgcgacaggctcgtggacaacgccttgagtggataggt

SEQ ID NO: 142 - protein, 14 aa, Artificial Sequence
  source: /note="Description of Artificial Sequence: Synthetic peptide"
WVRQAPGKGLEWVS

SEQ ID NO: 143 - DNA, 42 bp, Artificial Sequence
  source: /note="Description of Artificial Sequence: Synthetic oligonucleotide"
tgggtccgccaggctccagggaaggggctggagtgggtcagt

SEQ ID NO: 144 - protein, 32 aa, Artificial Sequence
  source: /note="Description of Artificial Sequence: Synthetic polypeptide"
RFTISRDDSKNTAYLQMNSLKTEDTAVYYCAR

SEQ ID NO: 145 - DNA, 96 bp, Artificial Sequence
  source: /note="Description of Artificial Sequence: Synthetic oligonucleotide"
agattcaccatctccagagatgattcaaagaacacggcgtatctgcaaatgaacagcctgaaaaccgaggacacggccgtgtattactgtgcaagg

SEQ ID NO: 146 - protein, 32 aa, Artificial Sequence
  source: /note="Description of Artificial Sequence: Synthetic polypeptide"
RVTITADKSTSTAYMELSSLRSEDTAVYYCAR

SEQ ID NO: 147 - DNA, 96 bp, Artificial Sequence
  source: /note="Description of Artificial Sequence: Synthetic oligonucleotide"
agagtcacgattaccgcggacaaatccacgagcacagcctacatggagctgagcagcctgagatctgaggacacggccgtgtattactgtgcaagg

SEQ ID NO: 148 - protein, 32 aa, Artificial Sequence
  source: /note="Description of Artificial Sequence: Synthetic polypeptide"
RVTISVDTSKNQFSLKLSSVTAADTAVYYCAR

SEQ ID NO: 149 - DNA, 96 bp, Artificial Sequence
  source: /note="Description of Artificial Sequence: Synthetic oligonucleotide"
agagtcaccatatcagtagacacgtccaagaaccagttctccctgaagctgagctctgtgaccgccgcggacacggctgtgtattactgtgcaagg

SEQ ID NO: 150 - protein, 32 aa, Artificial Sequence
  source: /note="Description of Artificial Sequence: Synthetic polypeptide"
RLTISKDTSKNQVVLTMTNMDPVDTATYYCAR

SEQ ID NO: 151 - DNA, 96 bp, Artificial Sequence
  source: /note="Description of Artificial Sequence: Synthetic oligonucleotide"
agactcaccatctccaaggacacctccaaaaaccaggtggtccttacaatgaccaacatggaccctgtggacacagccacgtattactgtgcaagg

SEQ ID NO: 152 - protein, 32 aa, Artificial Sequence
  source: /note="Description of Artificial Sequence: Synthetic polypeptide"
RFTISRDNSKNTLYLQMNSLRAEDTAVYYCAR

SEQ ID NO: 153 - DNA, 96 bp, Artificial Sequence
  source: /note="Description of Artificial Sequence: Synthetic oligonucleotide"
agattcaccatctccagagacaattccaagaacacgctgtatcttcaaatgaacagcctgagagccgaggacacggccgtgtattactgtgcaagg

SEQ ID NO: 154 - protein, 11 aa, Artificial Sequence
  source: /note="Description of Artificial Sequence: Synthetic peptide"
WGQGTTVTVSS

SEQ ID NO: 155 - DNA, 33 bp, Artificial Sequence
  source: /note="Description of Artificial Sequence: Synthetic oligonucleotide"
tggggccagggcaccaccgtgaccgtgtcctcc

SEQ ID NO: 156 - protein, 23 aa, Artificial Sequence
  source: /note="Description of Artificial Sequence: Synthetic peptide"
EIVLTQSPDFQSVTPKEKVTITC

SEQ ID NO: 157 - DNA, 69 bp, Artificial Sequence
  source: /note="Description of Artificial Sequence: Synthetic oligonucleotide"
gaaattgtgctgactcagtctccagactttcagtctgtgactccaaaggagaaagtcaccatcacctgc

SEQ ID NO: 158 - protein, 23 aa, Artificial Sequence
  source: /note="Description of Artificial Sequence: Synthetic peptide"
DVVMTQSPLSLPVTLGQPASISC

SEQ ID NO: 159 - DNA, 69 bp, Artificial Sequence
  source: /note="Description of Artificial Sequence: Synthetic oligonucleotide"
gatgttgtgatgactcagtctccactctccctgcccgtcacccttggacagccggcctccatctcctgc

SEQ ID NO: 160 - protein, 23 aa, Artificial Sequence
  source: /note="Description of Artificial Sequence: Synthetic peptide"
DIVMTQTPLSLPVTPGEPASISC

SEQ ID NO: 161 - DNA, 69 bp, Artificial Sequence
  source: /note="Description of Artificial Sequence: Synthetic oligonucleotide"
gatattgtgatgacccagactccactctccctgcccgtcacccctggagagccggcctccatctcctgc

SEQ ID NO: 162 - protein, 23 aa, Artificial Sequence
  source: /note="Description of Artificial Sequence: Synthetic peptide"
DIQMTQSPSSLSASVGDRVTITC

SEQ ID NO: 163 - DNA, 69 bp, Artificial Sequence
  source: /note="Description of Artificial Sequence: Synthetic oligonucleotide"
gacatccagatgacccagtctccatcctccctgtctgcatctgtaggagacagagtcaccatcacttgc

SEQ ID NO: 164 - protein, 23 aa, Artificial Sequence
  source: /note="Description of Artificial Sequence: Synthetic peptide"
EIVLTQSPATLSLSPGERATLSC

SEQ ID NO: 165 - DNA, 69 bp, Artificial Sequence
  source: /note="Description of Artificial Sequence: Synthetic oligonucleotide"
gaaattgtgttgacacagtctccagccaccctgtctttgtctccaggggaaagagccaccctctcctgc

SEQ ID NO: 166 - protein, 23 aa, Artificial Sequence
  source: /note="Description of Artificial Sequence: Synthetic peptide"
AIQLTQSPSSLSASVGDRVTITC

SEQ ID NO: 167 - DNA, 69 bp, Artificial Sequence
  source: /note="Description of Artificial Sequence: Synthetic oligonucleotide"
gccatccagttgacccagtctccatcctccctgtctgcatctgtaggagacagagtcaccatcacttgc

SEQ ID NO: 168 - protein, 15 aa, Artificial Sequence
  source: /note="Description of Artificial Sequence: Synthetic peptide"
WYQQKPGQAPRLLIY

SEQ ID NO: 169 - DNA, 45 bp, Artificial Sequence
  source: /note="Description of Artificial Sequence: Synthetic oligonucleotide"
tggtaccagcagaaacctggccaggctcccaggctcctcatctat

SEQ ID NO: 170 - protein, 15 aa, Artificial Sequence
  source: /note="Description of Artificial Sequence: Synthetic peptide"
WYLQKPGQSPQLLIY

SEQ ID NO: 171 - DNA, 45 bp, Artificial Sequence
  source: /note="Description of Artificial Sequence: Synthetic oligonucleotide"
tggtacctgcagaagccagggcagtctccacagctcctgatctat

SEQ ID NO: 172 - protein, 32 aa, Artificial Sequence
  source: /note="Description of Artificial Sequence: Synthetic polypeptide"
GVPSRFSGSGSGTEFTLTISSLQPDDFATYYC

SEQ ID NO: 173 - DNA, 96 bp, Artificial Sequence
  source: /note="Description of Artificial Sequence: Synthetic oligonucleotide"
ggggtcccatcaaggttcagcggcagtggatctgggacagaattcactctcaccatcagcagcctgcagcctgatgattttgcaacttattactgt

SEQ ID NO: 174 - protein, 32 aa, Artificial Sequence
  source: /note="Description of Artificial Sequence: Synthetic polypeptide"
GVPSRFSGSGSGTDFTFTISSLQPEDIATYYC

SEQ ID NO: 175 - DNA, 96 bp, Artificial Sequence
  source: /note="Description of Artificial Sequence: Synthetic oligonucleotide"
ggggtcccatcaaggttcagtggaagtggatctgggacagattttactttcaccatcagcagcctgcagcctgaagatattgcaacatattactgt

SEQ ID NO: 176 - protein, 32 aa, Artificial Sequence
  source: /note="Description of Artificial Sequence: Synthetic polypeptide"
GIPARFSGSGSGTEFTLTISSLQSEDFAVYYC

SEQ ID NO: 177 - DNA, 96 bp, Artificial Sequence
  source: /note="Description of Artificial Sequence: Synthetic oligonucleotide"
gggatcccagccaggttcagtggcagtgggtctgggacagagttcactctcaccatcagcagcctgcagtctgaagattttgcagtttattactgt

SEQ ID NO: 178 - protein, 32 aa, Artificial Sequence
  source: /note="Description of Artificial Sequence: Synthetic polypeptide"
GVPSRFSGSGSGTDFTLTISSLQPEDFATYYC

SEQ ID NO: 179 - DNA, 96 bp, Artificial Sequence
  source: /note="Description of Artificial Sequence: Synthetic oligonucleotide"
ggggtcccatcaaggttcagcggcagtggatctgggacagatttcactctcaccatcagcagcctgcagcctgaagattttgcaacttattactgt

SEQ ID NO: 180 - protein, 32 aa, Artificial Sequence
  source: /note="Description of Artificial Sequence: Synthetic polypeptide"
GVPDRFSGSGSGTDFTLKISRVEAEDVGVYYC

SEQ ID NO: 181 - DNA, 96 bp, Artificial Sequence
  source: /note="Description of Artificial Sequence: Synthetic oligonucleotide"
ggggtcccagacaggttcagtggcagtgggtcaggcactgatttcacactgaaaatcagcagggtggaggctgaggatgttggagtttattactgt

SEQ ID NO: 182 - protein, 32 aa, Artificial Sequence
  source: /note="Description of Artificial Sequence: Synthetic polypeptide"
GIPPRFSGSGYGTDFTLTINNIESEDAAYYFC

SEQ ID NO: 183 - DNA, 96 bp, Artificial Sequence
  source: /note="Description of Artificial Sequence: Synthetic oligonucleotide"
gggatcccacctcgattcagtggcagcgggtatggaacagattttaccctcacaattaataacatagaatctgaggatgctgcatattacttctgt

SEQ ID NO: 184 - protein, 32 aa, Artificial Sequence
  source: /note="Description of Artificial Sequence: Synthetic polypeptide"
GVPSRFSGSGSGTDFTFTISSLEAEDAATYYC

SEQ ID NO: 185 - DNA, 96 bp, Artificial Sequence
  source: /note="Description of Artificial Sequence: Synthetic oligonucleotide"
ggggtcccctcgaggttcagtggcagtggatctgggacagatttcacctttaccatcagtagcctggaagctgaagatgctgcaacatattactgt

SEQ ID NO: 186 - protein, 10 aa, Artificial Sequence
  source: /note="Description of Artificial Sequence: Synthetic peptide"
FGQGTKVEIK

SEQ ID NO: 187 - DNA, 30 bp, Artificial Sequence
  source: /note="Description of Artificial Sequence: Synthetic oligonucleotide"
ttcggccaagggaccaaggtggaaatcaaa

SEQ ID NO: 188 - protein, 327 aa, Artificial Sequence
  source: /note="Description of Artificial Sequence: Synthetic polypeptide"
ASTKGPSVFPLAPCSRSTSESTAALGCLVKDYFPEPVTVSWNSGALTSGVHTFPAVLQSSGLYSLSSVVTVPSSSLGTKTYTCNVDHKPSNTKVDKRVESKYGPPCPPCPAPEFLGGPSVFLFPPKPKDTLMISRTPEVTCVVVDVSQEDPEVQFNWYVDGVEVHNAKTKPREEQFNSTYRVVSVLTVLHQDWLNGKEYKCKVSNKGLPSSIEKTISKAKGQPREPQVYTLPPSQEEMTKNQVSLTCLVKGFYPSDIAVEWESNGQPENNYKTTPPVLDSDGSFFLYSRLTVDKSRWQEGNVFSCSVMHEALHNHYTQKSLSLSLGK

SEQ ID NO: 189 - protein, 107 aa, Artificial Sequence [sequence omitted]

SEQ ID NO: 190 - protein, 326 aa, Artificial Sequence
  source: /note="Description of Artificial Sequence: Synthetic polypeptide"
ASTKGPSVFPLAPCSRSTSESTAALGCLVKDYFPEPVTVSWNSGALTSGVHTFPAVLQSSGLYSLSSVVTVPSSSLGTKTYTCNVDHKPSNTKVDKRVESKYGPPCPPCPAPEFLGGPSVFLFPPKPKDTLMISRTPEVTCVVVDVSQEDPEVQFNWYVDGVEVHNAKTKPREEQFNSTYRVVSVLTVLHQDWLNGKEYKCKVSNKGLPSSIEKTISKAKGQPREPQVYTLPPSQEEMTKNQVSLTCLVKGFYPSDIAVEWESNGQPENNYKTTPPVLDSDGSFFLYSRLTVDKSRWQEGNVFSCSVMHEALHNHYTQKSLSLSLG

SEQ ID NO: 191 - protein, 330 aa, Artificial Sequence
  source: /note="Description of Artificial Sequence: Synthetic polypeptide"
ASTKGPSVFPLAPSSKSTSGGTAALGCLVKDYFPEPVTVSWNSGALTSGVHTFPAVLQSSGLYSLSSVVTVPSSSLGTQTYICNVNHKPSNTKVDKRVEPKSCDKTHTCPPCPAPELLGGPSVFLFPPKPKDTLMISRTPEVTCVVVDVSHEDPEVKFNWYVDGVEVHNAKTKPREEQYNSTYRVVSVLTVLHQDWLNGKEYKCKVSNKALPAPIEKTISKAKGQPREPQVYTLPPSREEMTKNQVSLTCLVKGFYPSDIAVEWESNGQPENNYKTTPPVLDSDGSFFLYSKLTVDKSRWQQGNVFSCSVMHEALHNHYTQKSLSLSPGK

SEQ ID NO: 192 - protein, 330 aa, Artificial Sequence
  source: /note="Description of Artificial Sequence: Synthetic polypeptide"
ASTKGPSVFPLAPSSKSTSGGTAALGCLVKDYFPEPVTVSWNSGALTSGVHTFPAVLQSSGLYSLSSVVTVPSSSLGTQTYICNVNHKPSNTKVDKRVEPKSCDKTHTCPPCPAPELLGGPSVFLFPPKPKDTLMISRTPEVTCVVVDVSHEDPEVKFNWYVDGVEVHNAKTKPREEQYASTYRVVSVLTVLHQDWLNGKEYKCKVSNKALPAPIEKTISKAKGQPREPQVYTLPPSREEMTKNQVSLTCLVKGFYPSDIAVEWESNGQPENNYKTTPPVLDSDGSFFLYSKLTVDKSRWQQGNVFSCSVMHEALHNHYTQKSLSLSPGK

SEQ ID NO: 193 - protein, 330 aa, Artificial Sequence
  source: /note="Description of Artificial Sequence: Synthetic polypeptide"
ASTKGPSVFPLAPSSKSTSGGTAALGCLVKDYFPEPVTVSWNSGALTSGVHTFPAVLQSSGLYSLSSVVTVPSSSLGTQTYICNVNHKPSNTKVDKRVEPKSCDKTHTCPPCPAPELLGGPSVFLFPPKPKDTLMISRTPEVTCVVVAVSHEDPEVKFNWYVDGVEVHNAKTKPREEQYNSTYRVVSVLTVLHQDWLNGKEYKCKVSNKALAAPIEKTISKAKGQPREPQVYTLPPSREEMTKNQVSLTCLVKGFYPSDIAVEWESNGQPENNYKTTPPVLDSDGSFFLYSKLTVDKSRWQQGNVFSCSVMHEALHNHYTQKSLSLSPGK

SEQ ID NO: 194 - protein, 330 aa, Artificial Sequence
  source: /note="Description of Artificial Sequence: Synthetic polypeptide"
ASTKGPSVFPLAPSSKSTSGGTAALGCLVKDYFPEPVTVSWNSGALTSGVHTFPAVLQSSGLYSLSSVVTVPSSSLGTQTYICNVNHKPSNTKVDKRVEPKSCDKTHTCPPCPAPEAAGGPSVFLFPPKPKDTLMISRTPEVTCVVVDVSHEDPEVKFNWYVDGVEVHNAKTKPREEQYNSTYRVVSVLTVLHQDWLNGKEYKCKVSNKALPAPIEKTISKAKGQPREPQVYTLPPSREEMTKNQVSLTCLVKGFYPSDIAVEWESNGQPENNYKTTPPVLDSDGSFFLYSKLTVDKSRWQQGNVFSCSVMHEALHNHYTQKSLSLSPGK

SEQ ID NO: 195 - protein, 10 aa, Artificial Sequence
  source: /note="Description of Artificial Sequence: Synthetic peptide"
GYTFTSYWMY

SEQ ID NO: 196 - DNA, 360 bp, Artificial Sequence
  source: /note="Description of Artificial Sequence: Synthetic polynucleotide"
gaagtgcagctggtgcagtctggcgccgaagtgaagaaacccggcgctaccgtgaagatctcctgcaaggtgtccggctacaccttcaccagctactggatgtactgggtgcgacaggctaccggccagggcctggaatggatgggcagaatcgaccccaactccggctccaccaagtacaacgagaagttcaagaaccgcgtgaccatcaccgccgacaagtccacctccaccgcctacatggaactgtcctccctgcggagcgaggacaccgccgtgtactactgcgccagagactaccggaagggcctgtacgccatggactattggggccagggcaccaccgtgaccgtgtcctct

SEQ ID NO: 197 - protein, 446 aa, Artificial Sequence; identical to SEQ ID NO: 96
  source: /note="Description of Artificial Sequence: Synthetic polypeptide"

SEQ ID NO: 198 - DNA, 1348 bp, Artificial Sequence
  source: /note="Description of Artificial Sequence: Synthetic polynucleotide"
gaagtgcagctggtgcagtctggcgccgaagtgaagaaacccggcgctaccgtgaagatctcctgcaaggtgtccggctacaccttcaccagctactggatgtactgggtgcgacaggctaccggccagggcctggaatggatgggcagaatcgaccccaactccggctccaccaagtacaacgagaagttcaagaaccgcgtgaccatcaccgccgacaagtccacctccaccgcctacatggaactgtcctccctgcggagcgaggacaccgccgtgtactactgcgccagagactaccggaagggcctgtacgccatggactattggggccagggcaccaccgtgaccgtgtcctctgcttccaccaagggcccaagcgtgttccccctggccccctgctccagaagcaccagcgagagcacagccgccctgggctgcctggtgaaggactacttccccgagcccgtgaccgtgtcctggaacagcggagccctgaccagcggcgtgcacaccttccccgccgtgctgcagagcagcggcctgtacagcctgagcagcgtggtgaccgtgcccagcagcagcctgggcaccaagacctacacctgtaacgtggaccacaagcccagcaacaccaaggtggacaagagggtggagagcaagtacggcccaccctgccccccctgcccagcccccgagttcctgggcggacccagcgtgttcctgttcccccccaagcccaaggacaccctgatgatcagcagaacccccgaggtgacctgtgtggtggtggacgtgtcccaggaggaccccgaggtccagttcaactggtacgtggacggcgtggaggtgcacaacgccaagaccaagcccagagaggagcagtttaacagcacctaccgggtggtgtccgtgctgaccgtgctgcaccaggactggctgaacggcaaagagtacaagtgtaaggtctccaacaagggcctgccaagcagcatcgaaaagaccatcagcaaggccaagggccagcctagagagccccaggtctacaccctgccacccagccaagaggagatgaccaagaaccaggtgtccctgacctgtctggtgaagggcttctacccaagcgacatcgccgtggagtgggagagcaacggccagcccgagaacaactacaagaccacccccccagtgctggacagcgacggcagcttcttcctgtacagcaggctgaccgtggacaagtccagatggcaggagggcaacgtctttagctgctccgtgatgcacgaggccctgcacaaccactacacccagaagagcctgagcctgtccctgggctgatgaattc

SEQ ID NO: 199 - DNA, 321 bp, Artificial Sequence
  source: /note="Description of Artificial Sequence: Synthetic polynucleotide"
gagatcgtgctgacccagtcccccgacttccagtccgtgacccccaaagaaaaagtgaccatcacatgcaaggcctcccaggacgtgggcaccgccgtggcttggtatctgcagaagcctggccagtcccctcagctgctgatctactgggcctctaccagacacaccggcgtgcccgacagattctccggctctggctctggcaccgacttcaccctgaagatctcccgggtggaagccgaggatgtgggcgtgtactactgccagcagtacaactcctaccccctgaccttcggccagggcaccaaggtggaaatcaag

SEQ ID NO: 200 - DNA, 652 bp, Artificial Sequence
  source: /note="Description of Artificial Sequence: Synthetic polynucleotide"
gagatcgtgctgacccagtcccccgacttccagtccgtgacccccaaagaaaaagtgaccatcacatgcaaggcctcccaggacgtgggcaccgccgtggcttggtatctgcagaagcctggccagtcccctcagctgctgatctactgggcctctaccagacacaccggcgtgcccgacagattctccggctctggctctggcaccgacttcaccctgaagatctcccgggtggaagccgaggatgtgggcgtgtactactgccagcagtacaactcctaccccctgaccttcggccagggcaccaaggtggaaatcaagcgtacggtggccgctcccagcgtgttcatcttccccccaagcgacgagcagctgaagagcggcaccgccagcgtggtgtgtctgctgaacaacttctaccccagggaggccaaggtgcagtggaaggtggacaacgccctgcagagcggcaacagccaggagagcgtcaccgagcaggacagcaaggactccacctacagcctgagcagcaccctgaccctgagcaaggccgactacgagaagcacaaggtgtacgcctgtgaggtgacccaccagggcctgtccagccccgtgaccaagagcttcaacaggggcgagtgctgatgaattc

SEQ ID NO: 201 - DNA, 360 bp, Artificial Sequence
  source: /note="Description of Artificial Sequence: Synthetic polynucleotide"
gaagtgcagctggtgcagtctggcgccgaagtgaagaagcctggcgagtccctgcggatctcctgcaagggctccggctacaccttcaccagctactggatgtactggatccggcagccccctggcaagggcctggaatggatcggcagaatcgaccccaactccggctccaccaagtacaacgagaagttcaagaaccgcgtgaccatcaccgccgacaagtccacctccaccgcctacatggaactgtcctccctgagatccgaggacaccgccgtgtactactgcgccagagactaccggaagggcctgtacgccatggactattggggccagggcaccaccgtgaccgtgtcctct

SEQ ID NO: 202 - DNA, 1348 bp, Artificial Sequence
  source: /note="Description of Artificial Sequence: Synthetic polynucleotide"
gaagtgcagctggtgcagtctggcgccgaagtgaagaagcctggcgagtccctgcggatctcctgcaagggctccggctacaccttcaccagctactggatgtactggatccggcagccccctggcaagggcctggaatggatcggcagaatcgaccccaactccggctccaccaagtacaacgagaagttcaagaaccgcgtgaccatcaccgccgacaagtccacctccaccgcctacatggaactgtcctccctgagatccgaggacaccgccgtgtactactgcgccagagactaccggaagggcctgtacgccatggactattggggccagggcaccaccgtgaccgtgtcctctgcttctaccaagggcccaagcgtgttccccctggccccctgctccagaagcaccagcgagagcacagccgccctgggctgcctggtgaaggactacttccccgagcccgtgaccgtgtcctggaacagcggagccctgaccagcggcgtgcacaccttccccgccgtgctgcagagcagcggcctgtacagcctgagcagcgtggtgaccgtgcccagcagcagcctgggcaccaagacctacacctgtaacgtggaccacaagcccagcaacaccaaggtggacaagagggtggagagcaagtacggcccaccctgccccccctgcccagcccccgagttcctgggcggacccagcgtgttcctgttcccccccaagcccaaggacaccctgatgatcagcagaacccccgaggtgacctgtgtggtggtggacgtgtcccaggaggaccccgaggtccagttcaactggtacgtggacggcgtggaggtgcacaacgccaagaccaagcccagagaggagcagtttaacagcacctaccgggtggtgtccgtgctgaccgtgctgcaccaggactggctgaacggcaaagagtacaagtgtaaggtctccaacaagggcctgccaagcagcatcgaaaagaccatcagcaaggccaagggccagcctagagagccccaggtctacaccctgccacccagccaagaggagatgaccaagaaccaggtgtccctgacctgtctggtgaagggcttctacccaagcgacatcgccgtggagtgggagagcaacggccagcccgagaacaactacaagaccacccccccagtgctggacagcgacggcagcttcttcctgtacagcaggctgaccgtggacaagtccagatggcaggagggcaacgtctttagctgctccgtgatgcacgaggccctgcacaaccactacacccagaagagcctgagcctgtccctgggctgatgaattc

SEQ ID NO: 203 - DNA, 321 bp, Artificial Sequence
  source: /note="Description of Artificial Sequence: Synthetic polynucleotide"
gagatcgtgctgacccagtcccccgacttccagtccgtgacccccaaagaaaaagtgaccatcacatgcaaggcctcccaggacgtgggcaccgccgtggcttggtatctgcagaagcctggccagtcccctcagctgctgatctactgggcctctaccagacacaccggcgtgccctccagattctccggctctggctctggcaccgactttaccttcaccatctccagcctgcagcccgaggatatcgccacctactactgccagcagtacaactcctaccccctgaccttcggccagggcaccaaggtggaaatcaag

SEQ ID NO: 204 - DNA, 652 bp, Artificial Sequence
  source: /note="Description of Artificial Sequence: Synthetic polynucleotide"
gagatcgtgctgacccagtcccccgacttccagtccgtgacccccaaagaaaaagtgaccatcacatgcaaggcctcccaggacgtgggcaccgccgtggcttggtatctgcagaagcctggccagtcccctcagctgctgatctactgggcctctaccagacacaccggcgtgccctccagattctccggctctggctctggcaccgactttaccttcaccatctccagcctgcagcccgaggatatcgccacctactactgccagcagtacaactcctaccccctgaccttcggccagggcaccaaggtggaaatcaagcgtacggtggccgctcccagcgtgttcatcttccccccaagcgacgagcagctgaagagcggcaccgccagcgtggtgtgtctgctgaacaacttctaccccagggaggccaaggtgcagtggaaggtggacaacgccctgcagagcggcaacagccaggagagcgtcaccgagcaggacagcaaggactccacctacagcctgagcagcaccctgaccctgagcaaggccgactacgagaagcacaaggtgtacgcctgtgaggtgacccaccagggcctgtccagccccgtgaccaagagcttcaacaggggcgagtgctgatgaattc

SEQ ID NO: 205 - DNA, 51 bp, Artificial Sequence
  source: /note="Description of Artificial Sequence: Synthetic oligonucleotide"
agaatcgaccccaactccggctccaccaagtacaacgagaagttcaagaac

SEQ ID NO: 206 - DNA, 33 bp, Artificial Sequence
  source: /note="Description of Artificial Sequence: Synthetic oligonucleotide"
gactaccggaagggcctgtacgccatggactat

SEQ ID NO: 207 - DNA, 21 bp, Artificial Sequence
  source: /note="Description of Artificial Sequence: Synthetic oligonucleotide"
ggctacaccttcaccagctac

SEQ ID NO: 208 - DNA, 18 bp, Artificial Sequence
  source: /note="Description of Artificial Sequence: Synthetic oligonucleotide"
gaccccaactccggctcc

SEQ ID NO: 209 - DNA, 33 bp, Artificial Sequence
  source: /note="Description of Artificial Sequence: Synthetic oligonucleotide"
aaggcctcccaggacgtgggcaccgccgtggct

SEQ ID NO: 210 - DNA, 21 bp, Artificial Sequence
  source: /note="Description of Artificial Sequence: Synthetic oligonucleotide"
tgggcctctaccagacacacc

SEQ ID NO: 211 - DNA, 27 bp, Artificial Sequence
  source: /note="Description of Artificial Sequence: Synthetic oligonucleotide"
cagcagtacaactcctaccccctgacc

SEQ ID NO: 212 - DNA, 21 bp, Artificial Sequence
  source: /note="Description of Artificial Sequence: Synthetic oligonucleotide"
tcccaggacgtgggcaccgcc

SEQ ID NO: 213 - DNA, 9 bp, Artificial Sequence
  source: /note="Description of Artificial Sequence: Synthetic oligonucleotide"
tgggcctct

SEQ ID NO: 214 - DNA, 18 bp, Artificial Sequence
  source: /note="Description of Artificial Sequence: Synthetic oligonucleotide"
tacaactcctaccccctg

SEQ ID NO: 215 - DNA, 75 bp, Artificial Sequence
  source: /note="Description of Artificial Sequence: Synthetic oligonucleotide"
gaagtgcagctggtgcagtcaggcgccgaagtgaagaagcccggcgagtcactgagaattagctgtaaaggttca

SEQ ID NO: 216 - DNA, 75 bp, Artificial Sequence
  source: /note="Description of Artificial Sequence: Synthetic oligonucleotide"
gaagtgcagctggtgcagtctggcgccgaagtgaagaagcctggcgagtccctgcggatctcctgcaagggctcc

SEQ ID NO: 217 - DNA, 75 bp, Artificial Sequence
  source: /note="Description of Artificial Sequence: Synthetic oligonucleotide"
gaagtgcagctggtgcagtctggcgccgaagtgaagaaacccggcgctaccgtgaagatctcctgcaaggtgtcc

SEQ ID NO: 218 - DNA, 75 bp, Artificial Sequence
  source: /note="Description of Artificial Sequence: Synthetic oligonucleotide"
gaagtgcagctggtgcagtcaggcgccgaagtgaagaaacccggcgctaccgtgaagattagctgtaaagtctca

SEQ ID NO: 219 - DNA, 42 bp, Artificial Sequence
  source: /note="Description of Artificial Sequence: Synthetic oligonucleotide"
tgggtgcgacaggctaccggccagggcctggaatggatgggc

SEQ ID NO: 220 - DNA, 42 bp, Artificial Sequence
  source: /note="Description of Artificial Sequence: Synthetic oligonucleotide"
tgggtccgacaggctaccggtcaaggcctggagtggatgggt

SEQ ID NO: 221 - DNA, 42 bp, Artificial Sequence
  source: /note="Description of Artificial Sequence: Synthetic oligonucleotide"
tgggtccgacaggccccagggcaaggcctggagtggatgggt

SEQ ID NO: 222 - DNA, 42 bp, Artificial Sequence
  source: /note="Description of Artificial Sequence: Synthetic oligonucleotide"
tggatccggcagccccctggcaagggcctggaatggatcggc

SEQ ID NO: 223 - DNA, 42 bp, Artificial Sequence
  source: /note="Description of Artificial Sequence: Synthetic oligonucleotide"
tgggtccgacaggctagagggcaaagactggagtggatcggt

SEQ ID NO: 224 - DNA, 96 bp, Artificial Sequence
  source: /note="Description of Artificial Sequence: Synthetic oligonucleotide"
cgcgtgaccatcaccgccgacaagtccacctccaccgcctacatggaactgtcctccctgcggagcgaggacaccgccgtgtactactgcgccaga

SEQ ID NO: 225 - DNA, 96 bp, Artificial Sequence
  source: /note="Description of Artificial Sequence: Synthetic oligonucleotide"
cgcgtgaccatcaccgccgacaagtccacctccaccgcctacatggaactgtcctccctgagatccgaggacaccgccgtgtactactgcgccaga

SEQ ID NO: 226 - DNA, 96 bp, Artificial Sequence
  source: /note="Description of Artificial Sequence: Synthetic oligonucleotide"
agagtgactatcaccgccgataagtctactagcaccgcctatatggaactgtctagcctgagatcagaggacaccgccgtctactactgcgctaga

SEQ ID NO: 227 - DNA, 96 bp, Artificial Sequence
  source: /note="Description of Artificial Sequence: Synthetic oligonucleotide"
agagtgactattagcgtggacacctctaagaatcagtttagcctgaagctgtctagcgtgaccgccgctgacaccgccgtctactactgcgctaga

SEQ ID NO: 228 - DNA, 96 bp, Artificial Sequence
  source: /note="Description of Artificial Sequence: Synthetic oligonucleotide"
aggttcactattagtagggataactctaagaacaccctgtacctgcagatgaatagcctgagagccgaggacaccgccgtctactactgcgctaga

SEQ ID NO: 229 - DNA, 33 bp, Artificial Sequence
  source: /note="Description of Artificial Sequence: Synthetic oligonucleotide"
tggggccagggcaccaccgtgaccgtgtcctct

SEQ ID NO: 230 - DNA, 33 bp, Artificial Sequence
  source: /note="Description of Artificial Sequence: Synthetic oligonucleotide"
tggggtcaaggcactaccgtgaccgtgtcttca

SEQ ID NO: 231 - DNA, 69 bp, Artificial Sequence
  source: /note="Description of Artificial Sequence: Synthetic oligonucleotide"
gagatcgtgctgacccagtcccccgacttccagtccgtgacccccaaagaaaaagtgaccatcacatgc

SEQ ID NO: 232 - DNA, 69 bp, Artificial Sequence
  source: /note="Description of Artificial Sequence: Synthetic oligonucleotide"
gagatcgtcctgactcagtcacccgactttcagtcagtgacccctaaagagaaagtcactatcacctgt

SEQ ID NO: 233 - DNA, 69 bp, Artificial Sequence
  source: /note="Description of Artificial Sequence: Synthetic oligonucleotide"
gacgtcgtgatgactcagtcacccctgagcctgcccgtgaccctggggcagcccgcctctattagctgt

SEQ ID NO: 234 - DNA, 69 bp, Artificial Sequence
  source: /note="Description of Artificial Sequence: Synthetic oligonucleotide"
gctattcagctgactcagtcacctagtagcctgagcgctagtgtgggcgatagagtgactatcacctgt

SEQ ID NO: 235 - DNA, 45 bp, Artificial Sequence
  source: /note="Description of Artificial Sequence: Synthetic oligonucleotide"
tggtatcagcagaagccagggcaagcccctagactgctgatctac

SEQ ID NO: 236 - DNA, 45 bp, Artificial Sequence
  source: /note="Description of Artificial Sequence: Synthetic oligonucleotide"
tggtatctgcagaagcctggccagtcccctcagctgctgatctac

SEQ ID NO: 237 - DNA, 45 bp, Artificial Sequence
  source: /note="Description of Artificial Sequence: Synthetic oligonucleotide"
tggtatctgcagaagcctggtcaatcacctcagctgctgatctac

SEQ ID NO: 238 - DNA, 96 bp, Artificial Sequence
  source: /note="Description of Artificial Sequence: Synthetic oligonucleotide"
ggcgtgccctctaggtttagcggtagcggtagtggcaccgagttcaccctgactatctcttcactgcagcccgacgacttcgctacctactactgt

SEQ ID NO: 239 - DNA, 96 bp, Artificial Sequence
  source: /note="Description of Artificial Sequence: Synthetic oligonucleotide"
ggcgtgccctctaggtttagcggtagcggtagtggcaccgacttcaccttcactatctcttcactgcagcccgaggatatcgctacctactactgt

SEQ ID NO: 240 - DNA, 96 bp, Artificial Sequence
  source: /note="Description of Artificial Sequence: Synthetic oligonucleotide"
ggcgtgccctccagattctccggctctggctctggcaccgactttaccttcaccatctccagcctgcagcccgaggatatcgccacctactactgc

SEQ ID NO: 241 - DNA, 96 bp, Artificial Sequence
  source: /note="Description of Artificial Sequence: Synthetic oligonucleotide"
ggcgtgcccgacagattctccggctctggctctggcaccgacttcaccctgaagatctcccgggtggaagccgaggatgtgggcgtgtactactgc

SEQ ID NO: 242 - DNA, 96 bp, Artificial Sequence
  source: /note="Description of Artificial Sequence: Synthetic oligonucleotide"
ggcgtgccctctaggtttagcggtagcggtagtggcaccgacttcaccttcactatctcttcactggaagccgaggacgccgctacctactactgt

SEQ ID NO: 243 - DNA, 30 bp, Artificial Sequence
  source: /note="Description of Artificial Sequence: Synthetic oligonucleotide"
ttcggccagggcaccaaggtggaaatcaag

SEQ ID NO: 244 - DNA, 30 bp, Artificial Sequence
  source: /note="Description of Artificial Sequence: Synthetic oligonucleotide"
ttcggtcaaggcactaaggtcgagattaag

SEQ ID NO: 245 - DNA, 33 bp, Artificial Sequence
  source: /note="Description of Artificial Sequence: Synthetic oligonucleotide"
aaggccagtcaggatgtgggtactgctgtagcc

SEQ ID NO: 246 - DNA, 21 bp, Artificial Sequence
  source: /note="Description of Artificial Sequence: Synthetic oligonucleotide"
tgggcatccacccggcacact

SEQ ID NO: 247 - protein, 447 aa, Artificial Sequence
  source: /note="Description of Artificial Sequence: Synthetic polypeptide"
EVQLVQSGAEVKKPGATVKISCKVSGYTFTSYWMYWVRQARGQRLEWIGRIDPNSGSTKYNEKFKNRFTISRDNSKNTLYLQMNSLRAEDTAVYYCARDYRKGLYAMDYWGQGTTVTVSSASTKGPSVFPLAPCSRSTSESTAALGCLVKDYFPEPVTVSWNSGALTSGVHTFPAVLQSSGLYSLSSVVTVPSSSLGTKTYTCNVDHKPSNTKVDKRVESKYGPPCPPCPAPEFLGGPSVFLFPPKPKDTLMISRTPEVTCVVVDVSQEDPEVQFNWYVDGVEVHNAKTKPREEQFNSTYRVVSVLTVLHQDWLNGKEYKCKVSNKGLPSSIEKTISKAKGQPREPQVYTLPPSQEEMTKNQVSLTCLVKGFYPSDIAVEWESNGQPENNYKTTPPVLDSDGSFFLYSRLTVDKSRWQEGNVFSCSVMHEALHNHYTQKSLSLSLGK

SEQ ID NO: 248 - protein, 98 aa, Artificial Sequence
  source: /note="Description of Artificial Sequence: Synthetic polypeptide"
QVQLQQPGAELVKPGASVKLSCKASGYTFTSYWMHWVKQRPGRGLEWIGRIDPNSGGTKYNEKFKSKATLTVDKPSSTAYMQLSSLTSEDSAVYYCAR

SEQ ID NO: 249 - protein, 107 aa, Artificial Sequence
  source: /note="Description of Artificial Sequence: Synthetic polypeptide"
DIVMTQSHKFMSTSVGDRVSITCKASQDVGTAVAWYQQKPGQSPKLLIYWASTRHTGVPDRFTGSGSGTDFTLTISNVQSEDLADYFCQQYSSYPLTFGAGSKLELK

SEQ ID NO: 250 - protein, 113 aa, Artificial Sequence
  source: /note="Description of Artificial Sequence: Synthetic polypeptide"
EVQLQQSGAELVKPGASVKLSCKASGYTFTSYWMYWVKQGPGRGLEWIGRIDPNSGSTKYNEKFKNKATLTVDKSSSTAYMQLSSLTSEDSAVYYCARDYRKGLYAMDYWGQG

SEQ ID NO: 251 - protein, 113 aa, Artificial Sequence
  source: /note="Description of Artificial Sequence: Synthetic polypeptide"
QVQLVQSGAEVKKPGASVKVSCKASGYTFTSYWMYWVRQATGQGLEWMGRIDPNSGSTKYNEKFKNRFTISRDDSKNTAYLQMNSLKTEDTAVYYCARDYRKGLYAMDYWGQG

SEQ ID NO: 252 - protein, 113 aa, Artificial Sequence
  source: /note="Description of Artificial Sequence: Synthetic polypeptide"
EVQLVQSGAEVKKPGESLRISCKGSGYTFTSYWMYWIRQPPGKGLEWIGRIDPNSGSTKYNEKFKNRVTITADKSTSTAYMELSSLRSEDTAVYYCARDYRKGLYAMDYWGQG

SEQ ID NO: 253 - protein, 113 aa, Artificial Sequence
  source: /note="Description of Artificial Sequence: Synthetic polypeptide"
EVQLVQSGAEVKKPGATVKISCKVSGYTFTSYWMYWVRQATGQGLEWMGRIDPNSGSTKYNEKFKNRVTITADKSTSTAYMELSSLRSEDTAVYYCARDYRKGLYAMDYWGQG

SEQ ID NO: 254 - protein, 113 aa, Artificial Sequence
  source: /note="Description of Artificial Sequence: Synthetic polypeptide"
EVQLVQSGAEVKKPGESLRISCKGSGYTFTSYWMYWVRQAPGQGLEWMGRIDPNSGSTKYNEKFKNRVTISVDTSKNQFSLKLSSVTAADTAVYYCARDYRKGLYAMDYWGQG

SEQ ID NO: 255 - protein, 113 aa, Artificial Sequence
  source: /note="Description of Artificial Sequence: Synthetic polypeptide"
QVQLVQSGAEVKKPGASVKVSCKASGYTFTSYWMYWIRQSPSRGLEWLGRIDPNSGSTKYNEKFKNRFTISRDDSKNTAYLQMNSLKTEDTAVYYCARDYRKGLYAMDYWGQG

SEQ ID NO: 256 - protein, 113 aa, Artificial Sequence
  source: /note="Description of Artificial Sequence: Synthetic polypeptide"
EVQLVQSGAEVKKPGESLRISCKGSGYTFTSYWMYWVRQARGQRLEWIGRIDPNSGSTKYNEKFKNRLTISKDTSKNQVVLTMTNMDPVDTATYYCARDYRKGLYAMDYWGQG

SEQ ID NO: 257 - protein, 113 aa, Artificial Sequence
  source: /note="Description of Artificial Sequence: Synthetic polypeptide"
EVQLVQSGAEVKKPGATVKISCKVSGYTFTSYWMYWIRQSPSRGLEWLGRIDPNSGSTKYNEKFKNRLTISKDTSKNQVVLTMTNMDPVDTATYYCARDYRKGLYAMDYWGQG

SEQ ID NO: 258 - protein, 113 aa, Artificial Sequence
  source: /note="Description of Artificial Sequence: Synthetic polypeptide"
QITLKESGPTLVKPTQTLTLTCTFSGYTFTSYWMYWVRQAPGKGLEWVSRIDPNSGSTKYNEKFKNRVTITADKSTSTAYMELSSLRSEDTAVYYCARDYRKGLYAMDYWGQG

SEQ ID NO: 259 - protein, 113 aa, Artificial Sequence
  source: /note="Description of Artificial Sequence: Synthetic polypeptide"
EVQLVQSGAEVKKPGATVKISCKVSGYTFTSYWMYWVRQARGQRLEWIGRIDPNSGSTKYNEKFKNRFTISRDNSKNTLYLQMNSLRAEDTAVYYCARDYRKGLYAMDYWGQG

SEQ ID NO: 260 - protein, 446 aa, Artificial Sequence
  source: /note="Description of Artificial Sequence: Synthetic polypeptide"
EVQLVQSGAEVKKPGESLRISCKGSGYTFTSYWMYWIRQPPGKGLEWIGRIDPNSGSTKYNEKFKNRVTITADKSTSTAYMELSSLRSEDTAVYYCARDYRKGLYAMDYWGQGTTVTVSSASTKGPSVFPLAPCSRSTSESTAALGCLVKDYFPEPVTVSWNSGALTSGVHTFPAVLQSSGLYSLSSVVTVPSSSLGTKTYTCNVDHKPSNTKVDKRVESKYGPPCPPCPAPEFLGGPSVFLFPPKPKDTLMISRTPEVTCVVVDVSQEDPEVQFNWYVDGVEVHNAKTKPREEQFNSTYRVVSVLTVLHQDWLNGKEYKCKVSNKGLPSSIEKTISKAKGQPREPQVYTLPPSQEEMTKNQVSLTCLVKGFYPSDIAVEWESNGQPENNYKTTPPVLDSDGSFFLYSRLTVDKSRWQEGNVFSCSVMHEALHNHYTQKSLSLSLG

SEQ ID NO: 261 - protein, 7 aa, Artificial Sequence
  source: /note="Description of Artificial Sequence: Synthetic peptide"
GYTFTTY

SEQ ID NO: 262 - protein, 6 aa, Artificial Sequence
  source: /note="Description of Artificial Sequence: Synthetic peptide"
YPGTGG

SEQ ID NO: 263 - protein, 8 aa, Artificial Sequence
  source: /note="Description of Artificial Sequence: Synthetic peptide"
WTTGTGAY

SEQ ID NO: 264 - protein, 13 aa, Artificial Sequence
  source: /note="Description of Artificial Sequence: Synthetic peptide"
SQSLLDSGNQKNF

SEQ ID NO: 265 - protein, 3 aa, Artificial Sequence
  source: /note="Description of Artificial Sequence: Synthetic peptide"
WAS

SEQ ID NO: 266 - protein, 6 aa, Artificial Sequence
  source: /note="Description of Artificial Sequence: Synthetic peptide"
DYSYPY

SEQ ID NO: 267 - protein, 5 aa, Artificial Sequence
  source: /note="Description of Artificial Sequence: Synthetic peptide"
TYWMH

SEQ ID NO: 268 - protein, 17 aa, Artificial Sequence
  source: /note="Description of Artificial Sequence: Synthetic peptide"
NIYPGTGGSNFDEKFKN

SEQ ID NO: 269 - protein, 17 aa, Artificial Sequence
  source: /note="Description of Artificial Sequence: Synthetic peptide"
KSSQSLLDSGNQKNFLT

SEQ ID NO: 270 - protein, 7 aa, Artificial Sequence
  source: /note="Description of Artificial Sequence: Synthetic peptide"
WASTRES

SEQ ID NO: 271 - protein, 9 aa, Artificial Sequence
  source: /note="Description of Artificial Sequence: Synthetic peptide"
QNDYSYPYT

SEQ ID NO: 272 - protein, 10 aa, Artificial Sequence
  source: /note="Description of Artificial Sequence: Synthetic peptide"
GYTFTTYWMH

SEQ ID NO: 273 - protein, 5 aa, Artificial Sequence
  source: /note="Description of Artificial Sequence: Synthetic peptide"
NYGMN

SEQ ID NO: 274 - protein, 7 aa, Artificial Sequence
  source: /note="Description of Artificial Sequence: Synthetic peptide"
GFTLTNY

SEQ ID NO: 275 - protein, 10 aa, Artificial Sequence
  source: /note="Description of Artificial Sequence: Synthetic peptide"
GFTLTNYGMN

SEQ ID NO: 276 - protein, 17 aa, Artificial Sequence
  source: /note="Description of Artificial Sequence: Synthetic peptide"
WINTDTGEPTYADDFKG

SEQ ID NO: 277 - protein, 16 aa, Artificial Sequence
  source: /note="Description of Artificial Sequence: Synthetic peptide"
NPPYYYGTNNAEAMDY

SEQ ID NO: 278 - protein, 11 aa, Artificial Sequence
  source: /note="Description of Artificial Sequence: Synthetic peptide"
SSSQDISNYLN

SEQ ID NO: 279 - protein, 7 aa, Artificial Sequence
  source: /note="Description of Artificial Sequence: Synthetic peptide"
YTSTLHL

SEQ ID NO: 280 - protein, 9 aa, Artificial Sequence
  source: /note="Description of Artificial Sequence: Synthetic peptide"
QQYYNLPWT

SEQ ID NO: 281 - protein, 6 aa, Artificial Sequence
  source: /note="Description of Artificial Sequence: Synthetic peptide"
NTDTGE

SEQ ID NO: 282 - protein, 7 aa, Artificial Sequence
  source: /note="Description of Artificial Sequence: Synthetic peptide"
SQDISNY

SEQ ID NO: 283 - protein, 3 aa, Artificial Sequence
  source: /note="Description of Artificial Sequence: Synthetic peptide"
YTS

SEQ ID NO: 284 - protein, 6 aa, Artificial Sequence
  source: /note="Description of Artificial Sequence: Synthetic peptide"
YYNLPW

SEQ ID NO: 285 - protein, 7 aa, Artificial Sequence
  source: /note="Description of Artificial Sequence: Synthetic peptide"
GYTFTSY

SEQ ID NO: 286 - protein, 6 aa, Artificial Sequence
  source: /note="Description of Artificial Sequence: Synthetic peptide"
YPGNGD

SEQ ID NO: 287 - protein, 9 aa, Artificial Sequence
  source: /note="Description of Artificial Sequence: Synthetic peptide"
VGGAFPMDY

SEQ ID NO: 288 - protein, 11 aa, Artificial Sequence
  source: /note="Description of Artificial Sequence: Synthetic peptide"
SESVEYYGTSL

SEQ ID NO: 289 - protein, 3 aa, Artificial Sequence
  source: /note="Description of Artificial Sequence: Synthetic peptide"
AAS

SEQ ID NO: 290 - protein, 6 aa, Artificial Sequence
  source: /note="Description of Artificial Sequence: Synthetic peptide"
SRKDPS

SEQ ID NO: 291 - protein, 5 aa, Artificial Sequence
  source: /note="Description of Artificial Sequence: Synthetic peptide"
SYNMH

SEQ ID NO: 292 - protein, 17 aa, Artificial Sequence
  source: /note="Description of Artificial Sequence: Synthetic peptide"
DIYPGNGDTSYNQKFKG

SEQ ID NO: 293 - protein, 15 aa, Artificial Sequence
  source: /note="Description of Artificial Sequence: Synthetic peptide"
RASESVEYYGTSLMQ

SEQ ID NO: 294 - protein, 7 aa, Artificial Sequence
  source: /note="Description of Artificial Sequence: Synthetic peptide"
AASNVES

SEQ ID NO: 295 - protein, 9 aa, Artificial Sequence
  source: /note="Description of Artificial Sequence: Synthetic peptide"
QQSRKDPST

SEQ ID NO: 296 - protein, 6 aa, Artificial Sequence
  source: /note="Description of Artificial Sequence: Synthetic peptide"
YPGSGD

SEQ ID NO: 297 - protein, 17 aa, Artificial Sequence
  source: /note="Description of Artificial Sequence: Synthetic peptide"
DIYPGSGDTSYNQKFKG

SEQ ID NO: 298 - protein, 6 aa, Artificial Sequence
  source: /note="Description of Artificial Sequence: Synthetic peptide"
YPGQGD

SEQ ID NO: 299 - protein, 17 aa, Artificial Sequence
  source: /note="Description of Artificial Sequence: Synthetic peptide"
DIYPGQGDTSYNQKFKG

SEQ ID NO: 300 - protein, 447 aa, Artificial Sequence
  source: /note="Description of Artificial Sequence: Synthetic polypeptide"
QVQLVQSGAEVKKPGSSVKVSCKASGYTFSSNVISWVRQAPGQGLEWMGGVIPIVDIANYAQRFKGRVTITADESTSTTYMELSSLRSEDTAVYYCASTLGLVLDAMDYWGQGTLVTVSSASTKGPSVFPLAPCSRSTSESTAALGCLVKDYFPEPVTVSWNSGALTSGVHTFPAVLQSSGLYSLSSVVTVPSSSLGTKTYTCNVDHKPSNTKVDKRVESKYGPPCPSCPAPEFLGGPSVFLFPPKPKDTLMISRTPEVTCVVVDVSQEDPEVQFNWYVDGVEVHNAKTKPREEQFNSTYRVVSVLTVLHQDWLNGKEYKCKVSNKGLPSSIEKTISKAKGQPREPQVYTLPPSQEEMTKNQVSLTCLVKGFYPSDIAVEWESNGQPENNYKTTPPVLDSDGSFFLYSRLTVDKSRWQEGNVFSCSVMHEALHNHYTQKSLSLSLGK

SEQ ID NO: 301 - protein, 215 aa, Artificial Sequence
  source: /note="Description of Artificial Sequence: Synthetic polypeptide"
ETVLTQSPGTLSLSPGERATLSCRASQSLGSSYLAWYQQKPGQAPRLLIYGASSRAPGIPDRFSGSGSGTDFTLTISRLEPEDFAVYYCQQYADSPITFGQGTRLEIKRTVAAPSVFIFPPSDEQLKSGTASVVCLLNNFYPREAKVQWKVDNALQSGNSQESVTEQDSKDSTYSLSSTLTLSKADYEKHKVYACEVTHQGLSSPVTKSFNRGEC

SEQ ID NO: 302 - protein, 121 aa, Artificial Sequence
  source: /note="Description of Artificial Sequence: Synthetic polypeptide"
QVQLVQSGAEVKKPGSSVKVSCKASGGTFSSYAISWVRQAPGQGLEWMGGIIPIFGTANYAQKFQGRVTITADESTSTAYMELSSLRSEDTAVYYCARGLWEVRALPSVYWGQGTLVTVSS

SEQ ID NO: 303 - protein, 109 aa, Artificial Sequence
  source: /note="Description of Artificial Sequence: Synthetic polypeptide"
SYELTQPPSVSVAPGQTARITCGANDIGSKSVHWYQQKAGQAPVLVVSEDIIRPSGIPERISGSNSGNTATLTISRVEAGDEADYYCQVWDRDSDQYVFGTGTKVTVLG

SEQ ID NO: 304 - protein, 440 aa, Artificial Sequence
  source: /note="Description of Artificial Sequence: Synthetic polypeptide"
QVQLVESGGGVVQPGRSLRLDCKASGITFSNSGMHWVRQAPGKGLEWVAVIWYDGSKRYYADSVKGRFTISRDNSKNTLFLQMNSLRAEDTAVYYCATNDDYWGQGTLVTVSSASTKGPSVFPLAPCSRSTSESTAALGCLVKDYFPEPVTVSWNSGALTSGVHTFPAVLQSSGLYSLSSVVTVPSSSLGTKTYTCNVDHKPSNTKVDKRVESKYGPPCPPCPAPEFLGGPSVFLFPPKPKDTLMISRTPEVTCVVVDVSQEDPEVQFNWYVDGVEVHNAKTKPREEQFNSTYRVVSVLTVLHQDWLNGKEYKCKVSNKGLPSSIEKTISKAKGQPREPQVYTLPPSQEEMTKNQVSLTCLVKGFYPSDIAVEWESNGQPENNYKTTPPVLDSDGSFFLYSRLTVDKSRWQEGNVFSCSVMHEALHNHYTQKSLSLSLGK

SEQ ID NO: 305 - protein, 214 aa, Artificial Sequence
  source: /note="Description of Artificial Sequence: Synthetic polypeptide"
EIVLTQSPATLSLSPGERATLSCRASQSVSSYLAWYQQKPGQAPRLLIYDASNRATGIPARFSGSGSGTDFTLTISSLEPEDFAVYYCQQSSNWPRTFGQGTKVEIKRTVAAPSVFIFPPSDEQLKSGTASVVCLLNNFYPREAKVQWKVDNALQSGNSQESVTEQDSKDSTYSLSSTLTLSKADYEKHKVYACEVTHQGLSSPVTKSFNRGEC

SEQ ID NO: 306 - protein, 447 aa, Artificial Sequence
  source: /note="Description of Artificial Sequence: Synthetic polypeptide"
QVQLVQSGVEVKKPGASVKVSCKASGYTFTNYYMYWVRQAPGQGLEWMGGINPSNGGTNFNEKFKNRVTLTTDSSTTTAYMELKSLQFDDTAVYYCARRDYRFDMGFDYWGQGTTVTVSSASTKGPSVFPLAPCSRSTSESTAALGCLVKDYFPEPVTVSWNSGALTSGVHTFPAVLQSSGLYSLSSVVTVPSSSLGTKTYTCNVDHKPSNTKVDKRVESKYGPPCPPCPAPEFLGGPSVFLFPPKPKDTLMISRTPEVTCVVVDVSQEDPEVQFNWYVDGVEVHNAKTKPREEQFNSTYRVVSVLTVLHQDWLNGKEYKCKVSNKGLPSSIEKTISKAKGQPREPQVYTLPPSQEEMTKNQVSLTCLVKGFYPSDIAVEWESNGQPENNYKTTPPVLDSDGSFFLYSRLTVDKSRWQEGNVFSCSVMHEALHNHYTQKSLSLSLGK

SEQ ID NO: 307 - protein, 218 aa, Artificial Sequence
  source: /note="Description of Artificial Sequence: Synthetic polypeptide"
EIVLTQSPATLSLSPGERATLSCRASKGVSTSGYSYLHWYQQKPGQAPRLLIYLASYLESGVPARFSGSGSGTDFTLTISSLEPEDFAVYYCQHSRDLPLTFGGGTKVEIKRTVAAPSVFIFPPSDEQLKSGTASVVCLLNNFYPREAKVQWKVDNALQSGNSQESVTEQDSKDSTYSLSSTLTLSKADYEKHKVYACEVTHQGLSSPVTKSFNRGEC

SEQ ID NO: 308 - protein, 118 aa, Artificial Sequence
  source: /note="Description of Artificial Sequence: Synthetic polypeptide"
EVQLLESGGGLVQPGGSLRLSCAASGFTFSSYIMMWVRQAPGKGLEWVSSIYPSGGITFYADKGRFTISRDNSKNTLYLQMNSLRAEDTAVYYCARIKLGTVTTVDYWGQGTLVTVSS

SEQ ID NO: 309 - protein, 110 aa, Artificial Sequence
  source: /note="Description of Artificial Sequence: Synthetic polypeptide"
QSALTQPASVSGSPGQSITISCTGTSSDVGGYNYVSWYQQHPGKAPKLMIYDVSNRPSGVSNRFSGSKSGNTASLTISGLQAEDEADYYCSSYTSSSTRVFGTGTKVTVL

SEQ ID NO: 310 - protein, 253 aa, Artificial Sequence [sequence omitted]

SEQ ID NO: 311 - protein, 263 aa, Artificial Sequence [sequence omitted]

SEQ ID NO: 312 - protein, 117 aa, Artificial Sequence
  source: /note="Description of Artificial Sequence: Synthetic polypeptide"
EVQLLESGGGLVQPGGSLRLSCAASGFTFSSYAMSWVRQAPGKGLEWVSGIGSYGGGTYYADSVKGRFTISRDNSKNTLYLQMNSLRAEDTAVYYCARYVNFGMDYWGQGTLVTVSS

SEQ ID NO: 313 - protein, 107 aa, Artificial Sequence
  source: /note="Description of Artificial Sequence: Synthetic polypeptide"
DIQMTQSPSSLSASVGDRVTITCRASQSISSYLNWYQQKPGKAPKLLIYAASSLQSGVPSRFSGSGSGTDFTLTISSLQPEDFATYYCQQYGRNPPTFGQGTKLEIK

SEQ ID NO: 314 - protein, 8 aa, Artificial Sequence
  source: /note="Description of Artificial Sequence: Synthetic peptide"
GFTFSSYA

SEQ ID NO: 315 - protein, 8 aa, Artificial Sequence
  source: /note="Description of Artificial Sequence: Synthetic peptide"
IGSYGGGT

SEQ ID NO: 316 - protein, 10 aa, Artificial Sequence
  source: /note="Description of Artificial Sequence: Synthetic peptide"
ARYVNFGMDY

SEQ ID NO: 317 - protein, 6 aa, Artificial Sequence
  source: /note="Description of Artificial Sequence: Synthetic peptide"
QSISSY

SEQ ID NO: 318 - protein, 9 aa, Artificial Sequence
  source: /note="Description of Artificial Sequence: Synthetic peptide"
QQYGRNPPT

SEQ ID NO: 319 - protein, 116 aa, Artificial Sequence
  source: /note="Description of Artificial Sequence: Synthetic polypeptide"
EVQLLESGGGLVQPGGSLRLSCAASGFTFSSYAMSWVRQAPGKGLEWVSAISGSGGSTYYADSVKGRFTISRDNSKNTLYLQMNSLRAEDTAVYYCARRVWGFDYWGQGTLVTVSS

SEQ ID NO: 320 - protein, 107 aa, Artificial Sequence
  source: /note="Description of Artificial Sequence: Synthetic polypeptide"
DIQMTQSPSSLSASVGDRVTITCRASQSISSYLNWYQQKPGKAPKLLIYAASSLQSGVPSRFSGSGSGTDFTLTISSLQPEDFATYYCQQYGVYPFTFGQGTKLEIK

SEQ ID NO: 321 - protein, 8 aa, Artificial Sequence
  source: /note="Description of Artificial Sequence: Synthetic peptide"
ISGSGGST

SEQ ID NO: 322 - protein, 9 aa, Artificial Sequence
  source: /note="Description of Artificial Sequence: Synthetic peptide"
ARRVWGFDY

SEQ ID NO: 323 - protein, 9 aa, Artificial Sequence
  source: /note="Description of Artificial Sequence: Synthetic peptide"
QQYGVYPFT

SEQ ID NO: 324 - protein, 128 aa, Artificial Sequence
  source: /note="Description of Artificial Sequence: Synthetic polypeptide"
  MOD_RES (120)..(120): Any amino acid
  MOD_RES (124)..(125): Any amino acid
EVRLQQSGADLVKPGASVKLSCASGFIIKATYMHWVRQRPEQGLEWIGRIDPANGEKYDPKFQVKAITADTSSSTAYLQLNSLTSDDTAVYYCARYAWYFDVWGAGTTVTVSSAKTTPPXVYPXXPGS

SEQ ID NO: 325 - protein, 127 aa, Artificial Sequence
  source: /note="Description of Artificial Sequence: Synthetic polypeptide"
DIQMTQSPASLSASVGDTVTITCRASENIYSFLAWYHQKQGRSPQLLVYHAKTLAEGVPSRFSGSGSGTQFSLKINSLQAEDFGSYYCQHYYGSPLTFGAGTKLEVKRADAAPTVSIFPPSSEELSL

SEQ ID NO: 326 - protein, 10 aa, Artificial Sequence
  source: /note="Description of Artificial Sequence: Synthetic peptide"
GFIIKATYMH

SEQ ID NO: 327 - protein, 17 aa, Artificial Sequence
  source: /note="Description of Artificial Sequence: Synthetic peptide"
RIDPANGETKYDPKFQV

SEQ ID NO: 328 - protein, 7 aa, Artificial Sequence
  source: /note="Description of Artificial Sequence: Synthetic peptide"
YAWYFDV

SEQ ID NO: 329 - protein, 11 aa, Artificial Sequence
  source: /note="Description of Artificial Sequence: Synthetic peptide"
RASENIYSFLA

SEQ ID NO: 330 - protein, 7 aa, Artificial Sequence
  source: /note="Description of Artificial Sequence: Synthetic peptide"
HAKTLAE

SEQ ID NO: 331 - protein, 9 aa, Artificial Sequence
  source: /note="Description of Artificial Sequence: Synthetic peptide"
QHYYGSPLT

SEQ ID NO: 332 - protein, 127 aa, Artificial Sequence [sequence omitted]

SEQ ID NO: 333 - protein, 127 aa, Artificial Sequence [sequence omitted]

SEQ ID NO: 334 - protein, 5 aa, Artificial Sequence
  source: /note="Description of Artificial Sequence: Synthetic peptide"
NYWMN

SEQ ID NO: 335 - protein, 17 aa, Artificial Sequence
  source: /note="Description of Artificial Sequence: Synthetic peptide"
AINQDGSEKYYVGSVKG

SEQ ID NO: 336 - protein, 18 aa, Artificial Sequence
  source: /note="Description of Artificial Sequence: Synthetic peptide"
DYYDILTDYYIHYWYFDL

SEQ ID NO: 337 - protein, 12 aa, Artificial Sequence
  source: /note="Description of Artificial Sequence: Synthetic peptide"
RASQSVSSSYLA

SEQ ID NO: 338 - protein, 7 aa, Artificial Sequence
  source: /note="Description of Artificial Sequence: Synthetic peptide"
GASSRAT

SEQ ID NO: 339 - protein, 446 aa, Artificial Sequence
  source: /note="Description of Artificial Sequence: Synthetic polypeptide"
EVQLVESGGDLVQPGGSLRLSCAASGFTFSSYWMSWVRQAPGKGLEWVANIKQDGSEKYYVDSVKGRFTISRDNAKNSLYLQMNSLRAEDTAVYYCARDRGSLYYWGQGTLVTVSSASTKGPSVFPLAPSSKSTSGGTAALGCLVKDYFPEPVTVSWNSGALTSGVHTFPAVLQSSGLYSLSSVVTVPSSSLGTQTYICNVNHKPSNTKVDKRVEPKSCDKTHTCPPCPAPELLGGPSVFLFPPKPKDTLMISRTPEVTCVVVDVSHEDPEVKFNWYVDGVEVHNAKTKPREEQYNSTYRVVSVLTVLHQDWLNGKEYKCKVSNKALPAPIEKTISKAKGQPREPQVYTLPPSREEMTKNQVSLTCLVKGFYPSDIAVEWESNGQPENNYKTTPPVLDSDGSFFLYSKLTVDKSRWQQGNVFSCSVMHEALHNHYTQKSLSLSPGK

SEQ ID NO: 340 - protein, 214 aa, Artificial Sequence
  source: /note="Description of Artificial Sequence: Synthetic polypeptide"
AIQLTQSPSSLSASVGDRVTITCRPSQGINWELAWYQQKPGKAPKLLIYDASSLEQGVPSRFSGSGSGTDFTLTISSLQPEDFATYYCQQFNSYPLTFGGGTKVEIKRTVAAPSVFIFPPSDEQLKSGTASVVCLLNNFYPREAKVQWKVDNALQSGNSQESVTEQDSKDSTYSLSSTLTLSKADYEKHKVYACEVTHQGLSSPVTKSFNRGEC

SEQ ID NO: 341 - protein, 119 aa, Artificial Sequence
  source: /note="Description of Artificial Sequence: Synthetic polypeptide"
QVQLVQSGAEVKKPGSSVKVSCKASGYSFTDYHIHWVRQAPGQGLEWMGVINPMYGTTDYNQRFKGRVTITADESTSTAYMELSSLRSEDTAVYYCARYDYFTGTGVYWGQGTLVTVSS

SEQ ID NO: 342 - protein, 112 aa, Artificial Sequence
  source: /note="Description of Artificial Sequence: Synthetic polypeptide"
DIVMTQTPLSLSVTPGQPASISCRSSRSLVHSRGNTYLHWYLQKPGQSPQLLIYKVSNRFIGVPDRFSGSGSGTDFTLKISRVEAEDVGVYYCSQSTHLPFTFGQGTKLEIK

SEQ ID NO: 343 - protein, 5 aa, Artificial Sequence
  source: /note="Description of Artificial Sequence: Synthetic peptide"
RYGIS

SEQ ID NO: 344 - protein, 17 aa, Artificial Sequence
  source: /note="Description of Artificial Sequence: Synthetic peptide"
WISTYSGNTNYAQKLQG

SEQ ID NO: 345 - protein, 7 aa, Artificial Sequence
  source: /note="Description of Artificial Sequence: Synthetic peptide"
RQLYFDY

SEQ ID NO: 346 - protein, 11 aa, Artificial Sequence
  source: /note="Description of Artificial Sequence: Synthetic peptide"
RASQSVSSNLA

SEQ ID NO: 347 - protein, 7 aa, Artificial Sequence
  source: /note="Description of Artificial Sequence: Synthetic peptide"
DASTRAT

SEQ ID NO: 348 - protein, 9 aa, Artificial Sequence
  source: /note="Description of Artificial Sequence: Synthetic peptide"
QQYDNWPLT

SEQ ID NO: 349 - protein, 137 aa, Artificial Sequence
  source: /note="Description of Artificial Sequence: Synthetic polypeptide"
MEFGLSWVFLVALLRGVQCQVQLVESGGGVVQPGRSLRLSCAASGFTFSVYGMNWVRQAPGKGLEWVAIIWYDGDNQYYADSVKGRFTISRDNSKNTLYLQMNGLRAEDTAVYYCARDLRTGPFDYWGQGTLVTVSS

SEQ ID NO: 350 - protein, 126 aa, Artificial Sequence
  source: /note="Description of Artificial Sequence: Synthetic polypeptide"
MLPSQLIGFLLLWVPASRGEIVLTQSPDFQSVTPKEKVTITCRASQSIGSSLHWYQQKPDQSPKLLIKYASQSFSGVPSRFSGSGSGTDFTLTINSLEAEDAAAYYCHQSSSLPFTFGPGTKVDIK

SEQ ID NO: 351 - protein, 12 aa, Artificial Sequence
  source: /note="Description of Artificial Sequence: Synthetic peptide"
GDSVSSNSAAWG

SEQ ID NO: 352 - protein, 18 aa, Artificial Sequence
  source: /note="Description of Artificial Sequence: Synthetic peptide"
RIYYRSKWYNSYAVSVKS

SEQ ID NO: 353 - protein, 12 aa, Artificial Sequence
  source: /note="Description of Artificial Sequence: Synthetic peptide"
RASQFISSSYLS

SEQ ID NO: 354 - protein, 11 aa, Artificial Sequence
  source: /note="Description of Artificial Sequence: Synthetic peptide"
LLIYGSSSRAT

SEQ ID NO: 355 - protein, 8 aa, Artificial Sequence
  source: /note="Description of Artificial Sequence: Synthetic peptide"
QQLYSSPM

SEQ ID NO: 356 - protein, 124 aa, Artificial Sequence
  source: /note="Description of Artificial Sequence: Synthetic polypeptide"
QVQLQQSGPGLVKPSQTLSLTCAISGDSVSSNSAAWGWIRQSPGRGLEWLGRIYYRSKWYNSYAVSVKSRITINPDTSKNQFSLQLNSVTPEDTAVYYCARYDWVPKIGVFDSWGQGTLVTVSS

SEQ ID NO: 357 - protein, 110 aa, Artificial Sequence
  source: /note="Description of Artificial Sequence: Synthetic polypeptide"
DIVLTQSPATLSLSPGERATLSCRASQFISSSYLSWYQQKPGQAPRLLIYGSSSRATGVPARFSGSGSGTDFTLTISSLEPEDFAVYYCQQLYSSPMTFGQGTKVEIKRT

SEQ ID NO: 358 - protein, 454 aa, Artificial Sequence
  source: /note="Description of Artificial Sequence: Synthetic polypeptide"
QVQLQQSGPGLVKPSQTLSLTCAISGDSVSSNSAAWGWIRQSPGRGLEWLGRIYYRSKWYNSYAVSVKSRITINPDTSKNQFSLQLNSVTPEDTAVYYCARYDWVPKIGVFDSWGQGTLVTVSSASTKGPSVFPLAPSSKSTSGGTAALGCLVKDYFPEPVTVSWNSGALTSGVHTFPAVLQSSGLYSLSSVVTVPSSSLGTQTYICNVNHKPSNTKVDKRVEPKSCDKTHTCPPCPAPELLGGPSVFLFPPKPKDTLMISRTPEVTCVVVDVSHEDPEVKFNWYVDGVEVHNAKTKPREEQYNSTYRVVSVLTVLHQDWLNGKEYKCKVSNKALPAPIEKTISKAKGQPREPQVYTLPPSREEMTKNQVSLTCLVKGFYPSDIAVEWESNGQPENNYKTTPPVLDSDGSFFLYSKLTVDKSRWQQGNVFSCSVMHEALHNHYTQKSLSLSPGK

SEQ ID NO: 359 - protein, 215 aa, Artificial Sequence
  source: /note="Description of Artificial Sequence: Synthetic polypeptide"
DIVLTQSPATLSLSPGERATLSCRASQFISSSYLSWYQQKPGQAPRLLIYGSSSRATGVPARFSGSGSGTDFTLTISSLEPEDFAVYYCQQLYSSPMTFGQGTKVEIKRTVAAPSVFIFPPSDEQLKSGTASVVCLLNNFYPREAKVQWKVDNALQSGNSQESVTEQDSKDSTYSLSSTLTLSKADYEKHKVYACEVTHQGLSSPVTKSFNRGEC

SEQ ID NO: 360 - protein, 4 aa, Artificial Sequence
  source: /note="Description of Artificial Sequence: Synthetic peptide"
RGDS

SEQ ID NO: 361 - protein, 9 aa, Artificial Sequence
  source: /note="Description of Artificial Sequence: Synthetic peptide"
QQYGSSPCT

SEQ ID NO: 362 - protein, 12 aa, Artificial Sequence
  source: /note="Description of Artificial Sequence: Synthetic peptide"
YDWVPKIGVFDS